European Patent Application EP 4 331 602 A1, published March 6, 2024. Title: A live attenuated SARS-CoV-2 and a vaccine made thereof. Applicant: Freie Universität Berlin. The sequence listing filed with the application follows.

SEQUENCE LISTING (56 sequences)

SEQ ID NO: 1 - RNA, 1482 nt, SARS-CoV-2
  source 1..1482: mol_type = genomic RNA
aaagatactactgaagcctttgaaaaaatggtttcactactttctgttttgctttccatgcagggtgctgtagacataaacaagctttgtgaagaaatgctggacaacagggcaaccttacaagctatagcctcagagtttagttcccttccatcatatgcagcttttgctactgctcaagaagcttatgagcaggctgttgctaatggtgattctgaagttgttcttaaaaagttgaagaagtctttgaatgtggctaaatctgaatttgaccgtgatgcagccatgcaacgtaagttggaaaagatggctgatcaagctatgacccaaatgtataaacaggctagatctgaggacaagagggcaaaagttactagtgctatgcagacaatgcttttcactatgcttagaaagttggataatgatgcactcaacaacattatcaacaatgcaagagatggttgtgttcccttgaacataatacctcttacaacagcagccaaactaatggttgtcataccagactataacacatataaaaatacgtgtgatggtacaacatttacttatgcatcagcattgtgggaaatccaacaggttgtagatgcagatagtaaaattgttcaacttagtgaaattagtatggacaattcacctaatttagcatggcctcttattgtaacagctttaagggccaattctgctgtcaaattacagaataatgagcttagtcctgttgcactacgacagatgtcttgtgctgccggtactacacaaactgcttgcactgatgacaatgcgttagcttactacaacacaacaaagggaggtaggtttgtacttgcactgttatccgatttacaggatttgaaatgggctagattccctaagagtgatggaactggtactatctatacagaactggaaccaccttgtaggtttgttacagacacacctaaaggtcctaaagtgaagtatttatactttattaaaggattaaacaacctaaatagaggtatggtacttggtagtttagctgccacagtacgtctacaagctggtaatgcaacagaagtgcctgccaattcaactgtattatctttctgtgcttttgctgtagatgctgctaaagcttacaaagattatctagctagtgggggacaaccaatcactaattgtgttaagatgttgtgtacacacactggtactggtcaggcaataacagttacaccggaagccaatatggatcaagaatcctttggtggtgcatcgtgttgtctgtactgccgttgccacatagatcatccaaatcctaaaggattttgtgacttaaaaggtaagtatgtacaaatacctacaacttgtgctaatgaccctgtgggttttacacttaaaaacacagtctgtaccgtctgcggtatgtggaaaggttatggctgtagttgtgatcaactccgcgaacccatgcttcagtcagctgat

SEQ ID NO: 2 - RNA, 1482 nt, synthetic construct
  source 1..1482: mol_type = other RNA
aaagatactaccgaagcattcgaaaaaatggttagtctgttatcggtactgttatctatgcaaggtgccgttgacattaataagttatgcgaagaaatgttagacaatagggctacattgcaagctatcgctagtgaatttagttcactaccatcatacgctgcattcgctacagctcaagaggcatacgagcaggcagtcgctaacggtgattccgaagtagtgcttaaaaaacttaaaaaatcacttaacgttgcgaaatccgaatttgatagggacgccgctatgcaacgtaagttagagaaaatggccgatcaggctatgacacaaatgtataaacaggctagatctgaggataaacgagctaaggttactagtgctatgcaaactatgttgtttactatgttacgtaaactcgataacgacgcacttaacaatataattaataacgctagagacggatgcgtaccacttaatattataccgttaactactgccgctaaattgatggtagttatacctgattataatacttataaaaatacatgtgacggtactacttttacatacgctagtgcattatgggaaatacaacaggtagtcgacgccgatagtaagatagtgcaattgtctgagatatctatggataatagtcctaatctcgcatggccattaatcgttaccgcattgcgtgctaactctgccgttaagttacagaataacgaattgtcaccagtcgcattgcgtcaaatgtcatgtgccgcaggtacgacacaaaccgcatgtacagacgataacgcattagcttattataatactactaagggaggtagattcgtactcgcactattatccgatttacaggatcttaaatgggctaggtttcctaaatctgacggtacaggtactatatataccgaactcgaacctccatgtagattcgttaccgatacacctaagggacctaaggttaagtatctatattttattaagggattgaataatcttaataggggtatggtattagggtcattagccgctacagttaggttgcaagccggtaacgctaccgaagtgccagctaatagtacggtactatctttttgtgcattcgcagttgacgctgctaaagcttataaagactatctagctagtggaggtcaacctattactaattgcgttaaaatgttatgtacacatacaggtacaggtcaagctattacggttacacctgaagctaatatggatcaggaatcattcggaggtgctagttgttgtctatattgtaggtgtcatatcgatcaccctaatcctaagggtttttgcgatcttaagggtaagtatgttcagatacctactacatgtgctaacgatcccgtaggttttacacttaaaaatacagtttgtacagtttgtggtatgtggaaaggttacggttgttcatgtgatcaattacgcgaacctatgttgcaatccgctgac

SEQ ID NO: 3 - RNA, 354 nt, SARS-CoV-2
  source 1..354: mol_type = genomic RNA
ttacgcgtatacgccaacttaggtgaacgtgtacgccaagctttgttaaaaacagtacaattctgtgatgccatgcgaaatgctggtattgttggtgtactgacattagataatcaagatctcaatggtaactggtatgatttcggtgatttcatacaaaccacgccaggtagtggagttcctgttgtagattcttattattcattgttaatgcctatattaaccttgaccagggctttaactgcagagtcacatgttgacactgacttaacaaagccttacattaagtgggatttgttaaaatatgacttcacggaagagaggttaaaactctttgaccgttattttaaatat

SEQ ID NO: 4 - RNA, 354 nt, synthetic construct
  source 1..354: mol_type = other RNA
ttacgcgtatacgctaacttaggcgaacgcgttagacaggcattacttaaaacagtgcaattttgtgacgctatgcgtaacgccggtatcgtaggtgtacttacacttgataatcaagaccttaacggtaattggtacgattttggtgattttatacagactacacctggttcaggtgtacccgtagtcgattcttattatagtctgttaatgcctatacttacacttacacgtgcattgactgccgaatctcacgttgatactgatctgactaagccttatattaaatgggatctgttaaaatacgattttacagaggaacgattgaaattgttcgataggtattttaagtat

SEQ ID NO: 5 - RNA, 2339 nt, SARS-CoV-2
  source 1..2339: mol_type = genomic RNA
aaagatactactgaagcctttgaaaaaatggtttcactactttctgttttgctttccatgcagggtgctgtagacataaacaagctttgtgaagaaatgctggacaacagggcaaccttacaagctatagcctcagagtttagttcccttccatcatatgcagcttttgctactgctcaagaagcttatgagcaggctgttgctaatggtgattctgaagttgttcttaaaaagttgaagaagtctttgaatgtggctaaatctgaatttgaccgtgatgcagccatgcaacgtaagttggaaaagatggctgatcaagctatgacccaaatgtataaacaggctagatctgaggacaagagggcaaaagttactagtgctatgcagacaatgcttttcactatgcttagaaagttggataatgatgcactcaacaacattatcaacaatgcaagagatggttgtgttcccttgaacataatacctcttacaacagcagccaaactaatggttgtcataccagactataacacatataaaaatacgtgtgatggtacaacatttacttatgcatcagcattgtgggaaatccaacaggttgtagatgcagatagtaaaattgttcaacttagtgaaattagtatggacaattcacctaatttagcatggcctcttattgtaacagctttaagggccaattctgctgtcaaattacagaataatgagcttagtcctgttgcactacgacagatgtcttgtgctgccggtactacacaaactgcttgcactgatgacaatgcgttagcttactacaacacaacaaagggaggtaggtttgtacttgcactgttatccgatttacaggatttgaaatgggctagattccctaagagtgatggaactggtactatctatacagaactggaaccaccttgtaggtttgttacagacacacctaaaggtcctaaagtgaagtatttatactttattaaaggattaaacaacctaaatagaggtatggtacttggtagtttagctgccacagtacgtctacaagctggtaatgcaacagaagtgcctgccaattcaactgtattatctttctgtgcttttgctgtagatgctgctaaagcttacaaagattatctagctagtgggggacaaccaatcactaattgtgttaagatgttgtgtacacacactggtactggtcaggcaataacagttacaccggaagccaatatggatcaagaatcctttggtggtgcatcgtgttgtctgtactgccgttgccacatagatcatccaaatcctaaaggattttgtgacttaaaaggtaagtatgtacaaatacctacaacttgtgctaatgaccctgtgggttttacacttaaaaacacagtctgtaccgtctgcggtatgtggaaaggttatggctgtagttgtgatcaactccgcgaacccatgcttcagtcagctgatgcacaatcgtttttaaacgggtttgcggtgtaagtgcagcccgtcttacaccgtgcggcacaggcactagtactgatgtcgtatacagggcttttgacatctacaatgataaagtagctggttttgctaaattcctaaaaactaattgttgtcgcttccaagaaaaggacgaagatgacaatttaattgattcttactttgtagttaagagacacactttctctaactaccaacatgaagaaacaatttataatttacttaaggattgtccagctgttgctaaacatgacttctttaagtttagaatagacggtgacatggtaccacatatatcacgtcaacgtcttactaaatacacaatggcagacctcgtctatgctttaaggcattttgatgaaggtaattgtgacacattaaaagaaatacttgtcacatacaattgttgtgatgatgattatttcaataaaaaggactggtatgattttgtagaaaacccagatatattacgcgtatacgccaacttaggtgaacgtgtacgccaagctttgttaaaaacagtacaattctgtgatgccatgcgaaatgctggtattgttggtgtactgacattagataatcaagatctcaatggtaactggtatgatttcggtgatttcatacaaaccacgccaggtagtggagttcctgttgtagattcttattattcattgttaatgcctatattaaccttgaccagggctttaactgcagagtcacatgttgacactgacttaacaaagccttacattaagtgggatttgttaaaatatgacttcacggaagagaggttaaaactctttgaccgttattttaaatat

SEQ ID NO: 6 - RNA, 2339 nt, synthetic construct
  source 1..2339: mol_type = other RNA
aaagatactaccgaagcattcgaaaaaatggttagtctgttatcggtactgttatctatgcaaggtgccgttgacattaataagttatgcgaagaaatgttagacaatagggctacattgcaagctatcgctagtgaatttagttcactaccatcatacgctgcattcgctacagctcaagaggcatacgagcaggcagtcgctaacggtgattccgaagtagtgcttaaaaaacttaaaaaatcacttaacgttgcgaaatccgaatttgatagggacgccgctatgcaacgtaagttagagaaaatggccgatcaggctatgacacaaatgtataaacaggctagatctgaggataaacgagctaaggttactagtgctatgcaaactatgttgtttactatgttacgtaaactcgataacgacgcacttaacaatataattaataacgctagagacggatgcgtaccacttaatattataccgttaactactgccgctaaattgatggtagttatacctgattataatacttataaaaatacatgtgacggtactacttttacatacgctagtgcattatgggaaatacaacaggtagtcgacgccgatagtaagatagtgcaattgtctgagatatctatggataatagtcctaatctcgcatggccattaatcgttaccgcattgcgtgctaactctgccgttaagttacagaataacgaattgtcaccagtcgcattgcgtcaaatgtcatgtgccgcaggtacgacacaaaccgcatgtacagacgataacgcattagcttattataatactactaagggaggtagattcgtactcgcactattatccgatttacaggatcttaaatgggctaggtttcctaaatctgacggtacaggtactatatataccgaactcgaacctccatgtagattcgttaccgatacacctaagggacctaaggttaagtatctatattttattaagggattgaataatcttaataggggtatggtattagggtcattagccgctacagttaggttgcaagccggtaacgctaccgaagtgccagctaatagtacggtactatctttttgtgcattcgcagttgacgctgctaaagcttataaagactatctagctagtggaggtcaacctattactaattgcgttaaaatgttatgtacacatacaggtacaggtcaagctattacggttacacctgaagctaatatggatcaggaatcattcggaggtgctagttgttgtctatattgtaggtgtcatatcgatcaccctaatcctaagggtttttgcgatcttaagggtaagtatgttcagatacctactacatgtgctaacgatcccgtaggttttacacttaaaaatacagtttgtacagtttgtggtatgtggaaaggttacggttgttcatgtgatcaattacgcgaacctatgttgcaatccgctgacgcacaatcgtttttaaacgggtttgcggtgtaagtgcagcccgtcttacaccgtgcggcacaggcactagtactgatgtcgtatacagggcttttgacatctacaatgataaagtagctggttttgctaaattcctaaaaactaattgttgtcgcttccaagaaaaggacgaagatgacaatttaattgattcttactttgtagttaagagacacactttctctaactaccaacatgaagaaacaatttataatttacttaaggattgtccagctgttgctaaacatgacttctttaagtttagaatagacggtgacatggtaccacatatatcacgtcaacgtcttactaaatacacaatggcagacctcgtctatgctttaaggcattttgatgaaggtaattgtgacacattaaaagaaatacttgtcacatacaattgttgtgatgatgattatttcaataaaaaggactggtatgattttgtagaaaacccagatatattacgcgtatacgctaacttaggcgaacgcgttagacaggcattacttaaaacagtgcaattttgtgacgctatgcgtaacgccggtatcgtaggtgtacttacacttgataatcaagaccttaacggtaattggtacgattttggtgattttatacagactacacctggttcaggtgtacccgtagtcgattcttattatagtctgttaatgcctatacttacacttacacgtgcattgactgccgaatctcacgttgatactgatctgactaagccttatattaaatgggatctgttaaaatacgattttacagaggaacgattgaaattgttcgataggtattttaagtat

SEQ ID NO: 7 - RNA, 1146 nt, SARS-CoV-2
  source 1..1146: mol_type = genomic RNA
ggtttacatctactgattggactagctaaacgttttaaggaatcaccttttgaattagaagattttattcctatggacagtacagttaaaaactatttcataacagatgcgcaaacaggttcatctaagtgtgtgtgttctgttattgatttattacttgatgattttgttgaaataataaaatcccaagatttatctgtagtttctaaggttgtcaaagtgactattgactatacagaaatttcatttatgctttggtgtaaagatggccatgtagaaacattttacccaaaattacaatctagtcaagcgtggcaaccgggtgttgctatgcctaatctttacaaaatgcaaagaatgctattagaaaagtgtgaccttcaaaattatggtgatagtgcaacattacctaaaggcataatgatgaatgtcgcaaaatatactcaactgtgtcaatatttaaacacattaacattagctgtaccctataatatgagagttatacattttggtgctggttctgataaaggagttgcaccaggtacagctgttttaagacagtggttgcctacgggtacgctgcttgtcgattcagatcttaatgactttgtctctgatgcagattcaactttgattggtgattgtgcaactgtacatacagctaataaatgggatctcattattagtgatatgtacgaccctaagactaaaaatgttacaaaagaaaatgactctaaagagggttttttcacttacatttgtgggtttatacaacaaaagctagctcttggaggttccgtggctataaagataacagaacattcttggaatgctgatctttataagctcatgggacacttcgcatggtggacagcctttgttactaatgtgaatgcgtcatcatctgaagcatttttaattggatgtaattatcttggcaaaccacgcgaacaaatagatggttatgtcatgcatgcaaattacatattttggaggaatacaaatccaattcagttgtcttcctattctttatttgacatgagtaaatttccccttaaattaaggggtactgctgttatgtctttaaaagaaggtcaaatcaatgatatgattttatctcttcttagtaaaggtagacttataatt

SEQ ID NO: 8 - RNA, 1146 nt, synthetic construct
  source 1..1146: mol_type = other RNA
gggttacatttacttatagggttagctaaaagatttaaagaatcaccattcgaactcgaagactttatacctatggatagtacggttaagaattattttattactgacgctcaaaccggttcatctaaatgcgtttgttcagttatagacttactgttagacgattttgtcgaaattattaagtctcaggatctatcagtcgtatctaaagtcgttaaggttacaatcgattatactgagatatcttttatgttatggtgtaaagacggtcacgttgagactttttatcctaaattgcaatctagtcaagcttggcaacccggtgtcgctatgcctaatctatataaaatgcaacgtatgttactcgaaaaatgcgatttacagaattacggtgattccgctacattgcctaaaggtattatgatgaatgtcgctaaatatacacaattgtgtcaatatcttaatacacttacacttgcagttccatataatatgagagtgatacattttggcgcaggatctgataagggagtcgcaccaggtactgccgtacttagacaatggttacctacaggtacactgttagtcgattccgatcttaacgattttgtttctgacgctgattctacacttataggcgattgtgctacagtgcataccgctaataaatgggatcttattatatccgatatgtacgatcctaaaactaaaaacgttactaaggaaaacgattctaaagagggtttttttacttatatttgtggttttatacagcaaaaattagcgttaggcggatccgttgcgattaagattaccgaacatagttggaatgctgatctatataagcttatgggtcatttcgcatggtggactgcattcgttacgaatgttaacgcttctagttccgaagcttttttaatcggatgtaattatttaggtaagcctagggaacagattgacggatacgttatgcatgctaattatattttttggcgtaatactaatcctattcaattgtctagttattcattattcgatatgtctaaatttccacttaaacttaggggtactgccgttatgtcacttaaggaaggtcaaattaacgatatgatactatcattgttatctaaaggtagattgattata

SEQ ID NO: 9 - RNA, 999 nt, SARS-CoV-2
  source 1..999: mol_type = genomic RNA
aaccaatttaatagtgctattggcaaaattcaagactcactttcttccacagcaagtgcacttggaaaacttcaagatgtggtcaaccaaaatgcacaagctttaaacacgcttgttaaacaacttagctccaattttggtgcaatttcaagtgttttaaatgatatcctttcacgtcttgacaaagttgaggctgaagtgcaaattgataggttgatcacaggcagacttcaaagtttgcagacatatgtgactcaacaattaattagagctgcagaaatcagagcttctgctaatcttgctgctactaaaatgtcagagtgtgtacttggacaatcaaaaagagttgatttttgtggaaagggctatcatcttatgtccttccctcagtcagcacctcatggtgtagtcttcttgcatgtgacttatgtccctgcacaagaaaagaacttcacaactgctcctgccatttgtcatgatggaaaagcacactttcctcgtgaaggtgtctttgtttcaaatggcacacactggtttgtaacacaaaggaatttttatgaaccacaaatcattactacagacaacacatttgtgtctggtaactgtgatgttgtaataggaattgtcaacaacacagtttatgatcctttgcaacctgaattagactcattcaaggaggagttagataaatattttaagaatcatacatcaccagatgttgatttaggtgacatctctggcattaatgcttcagttgtaaacattcaaaaagaaattgaccgcctcaatgaggttgccaagaatttaaatgaatctctcatcgatctccaagaacttggaaagtatgagcagtatataaaatggccatggtacatttggctaggttttatagctggcttgattgccatagtaatggtgacaattatgctttgctgtatgaccagttgctgtagttgtctcaagggctgttgttcttgtggatcctgctgcaaatttgat

SEQ ID NO: 10 - RNA, 999 nt, synthetic construct
  source 1..999: mol_type = other RNA
aaccaatttaattccgctataggtaagattcaagactcattgtctagtaccgctagtgcattaggtaagttgcaagacgtcgttaaccaaaacgctcaagcacttaatacacttgttaagcaattgtctagtaattttggcgctattagttcagtgcttaacgatattctatcacgtcttgataaagtcgaagccgaagtgcaaatcgatagattgattaccggtagattgcaatctcttcaaacttatgttacacaacaattgattagggctgccgaaattagggctagtgctaatctcgcagctactaaaatgtctgaatgcgtactcggtcaatctaaacgtgtcgatttttgcggtaagggatatcatcttatgtcttttccacaatccgcaccacatggagtggtttttttacacgttacatacgttccagctcaggaaaaaaattttactaccgcaccagctatttgtcatgacggtaaggcacattttcctagagagggagtattcgtttctaacggtacacattggttcgttacacaacgtaatttttacgagccacaaattattactactgataatacattcgttagcggtaattgcgacgtagtgataggtatagttaataatacagtttacgatccattgcaacctgaactcgattcttttaaagaggaactcgataagtattttaaaaaccatacatcacctgacgttgacttaggcgatatttccggtattaacgctagcgtagttaatattcaaaaagaaattgatagacttaacgaagtcgctaaaaaccttaacgaatcacttatcgatcttcaagagttaggtaagtatgagcaatatattaaatggccttggtatatttggttagggtttatagccggtcttatcgcaatcgttatggttacaattatgttatgttgtatgacatcatgttgttcatgtcttaagggatgttgttcatgcggatcatgttgtaaatttgac

SEQ ID NO: 11 - protein, 494 aa, SARS-CoV-2
KDTTEAFEKMVSLLSVLLSMQGAVDINKLCEEMLDNRATLQAIASEFSSLPSYAAFATAQEAYEQAVANGDSEVVLKKLKKSLNVAKSEFDRDAAMQRKLEKMADQAMTQMYKQARSEDKRAKVTSAMQTMLFTMLRKLDNDALNNIINNARDGCVPLNIIPLTTAAKLMVVIPDYNTYKNTCDGTTFTYASALWEIQQVVDADSKIVQLSEISMDNSPNLAWPLIVTALRANSAVKLQNNELSPVALRQMSCAAGTTQTACTDDNALAYYNTTKGGRFVLALLSDLQDLKWARFPKSDGTGTIYTELEPPCRFVTDTPKGPKVKYLYFIKGLNNLNRGMVLGSLAATVRLQAGNATEVPANSTVLSFCAFAVDAAKAYKDYLASGGQPITNCVKMLCTHTGTGQAITVTPEANMDQESFGGASCCLYCRCHIDHPNPKGFCDLKGKYVQIPTTCANDPVGFTLKNTVCTVCGMWKGYGCSCDQLREPMLQSAD

SEQ ID NO: 12 - protein, 118 aa, SARS-CoV-2
LRVYANLGERVRQALLKTVQFCDAMRNAGIVGVLTLDNQDLNGNWYDFGDFIQTTPGSGVPVVDSYYSLLMPILTLTRALTAESHVDTDLTKPYIKWDLLKYDFTEERLKLFDRYFKY

SEQ ID NO: 13 - protein, 382 aa, SARS-CoV-2
GLHLLIGLAKRFKESPFELEDFIPMDSTVKNYFITDAQTGSSKCVCSVIDLLLDDFVEIIKSQDLSVVSKVVKVTIDYTEISFMLWCKDGHVETFYPKLQSSQAWQPGVAMPNLYKMQRMLLEKCDLQNYGDSATLPKGIMMNVAKYTQLCQYLNTLTLAVPYNMRVIHFGAGSDKGVAPGTAVLRQWLPTGTLLVDSDLNDFVSDADSTLIGDCATVHTANKWDLIISDMYDPKTKNVTKENDSKEGFFTYICGFIQQKLALGGSVAIKITEHSWNADLYKLMGHFAWWTAFVTNVNASSSEAFLIGCNYLGKPREQIDGYVMHANYIFWRNTNPIQLSSYSLFDMSKFPLKLRGTAVMSLKEGQINDMILSLLSKGRLII

SEQ ID NO: 14 - protein, 333 aa, SARS-CoV-2
NQFNSAIGKIQDSLSSTASALGKLQDVVNQNAQALNTLVKQLSSNFGAISSVLNDILSRLDKVEAEVQIDRLITGRLQSLQTYVTQQLIRAAEIRASANLAATKMSECVLGQSKRVDFCGKGYHLMSFPQSAPHGVVFLHVTYVPAQEKNFTTAPAICHDGKAHFPREGVFVSNGTHWFVTQRNFYEPQIITTDNTFVSGNCDVVIGIVNNTVYDPLQPELDSFKEELDKYFKNHTSPDVDLGDISGINASVVNIQKEIDRLNEVAKNLNESLIDLQELGKYEQYIKWPWYIWLGFIAGLIAIVMVTIMLCCMTSCCSCLKGCCSCGSCCKFD

SEQ ID NO: 15 - RNA, 2943 nt, synthetic construct
  source 1..2943: mol_type = other RNA
tcaaccgctactttagactgactcttggtgtttatgattacttagtttctacacaggagtttagatatatgaattcacagggactactcccacccaagaatagcatagatgccttcaaactcaacattaaattgttgggtgttggtggcaaaccttgtatcaaagtagccactgtacagtctaaaatgtcagatgtaaagtgcacatcagtagtcttactctcagttttgcaacaactcagagtagaatcatcatctaaattgtgggctcaatgtgtccagttacacaatgacattctcttagctaaagatactaccgaagcattcgaaaaaatggttagtctgttatcggtactgttatctatgcaaggtgccgttgacattaataagttatgcgaagaaatgttagacaatagggctacattgcaagctatcgctagtgaatttagttcactaccatcatacgctgcattcgctacagctcaagaggcatacgagcaggcagtcgctaacggtgattccgaagtagtgcttaaaaaacttaaaaaatcacttaacgttgcgaaatccgaatttgatagggacgccgctatgcaacgtaagttagagaaaatggccgatcaggctatgacacaaatgtataaacaggctagatctgaggataaacgagctaaggttactagtgctatgcaaactatgttgtttactatgttacgtaaactcgataacgacgcacttaacaatataattaataacgctagagacggatgcgtaccacttaatattataccgttaactactgccgctaaattgatggtagttatacctgattataatacttataaaaatacatgtgacggtactacttttacatacgctagtgcattatgggaaatacaacaggtagtcgacgccgatagtaagatagtgcaattgtctgagatatctatggataatagtcctaatctcgcatggccattaatcgttaccgcattgcgtgctaactctgccgttaagttacagaataacgaattgtcaccagtcgcattgcgtcaaatgtcatgtgccgcaggtacgacacaaaccgcatgtacagacgataacgcattagcttattataatactactaagggaggtagattcgtactcgcactattatccgatttacaggatcttaaatgggctaggtttcctaaatctgacggtacaggtactatatataccgaactcgaacctccatgtagattcgttaccgatacacctaagggacctaaggttaagtatctatattttattaagggattgaataatcttaataggggtatggtattagggtcattagccgctacagttaggttgcaagccggtaacgctaccgaagtgccagctaatagtacggtactatctttttgtgcattcgcagttgacgctgctaaagcttataaagactatctagctagtggaggtcaacctattactaattgcgttaaaatgttatgtacacatacaggtacaggtcaagctattacggttacacctgaagctaatatggatcaggaatcattcggaggtgctagttgttgtctatattgtaggtgtcatatcgatcaccctaatcctaagggtttttgcgatcttaagggtaagtatgttcagatacctactacatgtgctaacgatcccgtaggttttacacttaaaaatacagtttgtacagtttgtggtatgtggaaaggttacggttgttcatgtgatcaattacgcgaacctatgttgcaatccgctgacgcacaatcgtttttaaacgggtttgcggtgtaagtgcagcccgtcttacaccgtgcggcacaggcactagtactgatgtcgtatacagggcttttgacatctacaatgataaagtagctggttttgctaaattcctaaaaactaattgttgtcgcttccaagaaaaggacgaagatgacaatttaattgattcttactttgtagttaagagacacactttctctaactaccaacatgaagaaacaatttataatttacttaaggattgtccagctgttgctaaacatgacttctttaagtttagaatagacggtgacatggtaccacatatatcacgtcaacgtcttactaaatacacaatggcagacctcgtctatgctttaaggcattttgatgaaggtaattgtgacacattaaaagaaatacttgtcacatacaattgttgtgatgatgattatttcaataaaaaggactggtatgattttgtagaaaacccagatatattacgcgtatacgctaacttaggcgaacgcgttagacaggcattacttaaaacagtgcaattttgtgacgctatgcgtaacgccggtatcgtaggtgtacttacacttgataatcaagaccttaacggtaattggtacgattttggtgattttatacagactacacctggttcaggtgtacccgtagtcgattcttattatagtctgttaatgcctatacttacacttacacgtgcattgactgccgaatctcacgttgatactgatctgactaagccttatattaaatgggatctgttaaaatacgattttacagaggaacgattgaaattgttcgataggtattttaagtattgggatcagacataccacccaaattgtgttaactgtttggatgacagatgcattctgcattgtgcaaactttaatgttttattctctacagtgttcccacctacaagttttggaccactagtgagaaaaatatttgttgatggtgttccatttgtagtttcaactggataccacttcagagagctaggtgttgtacataatcaggatgtaaacttacatagctctagacttagttttaaggaattacttgtgtatgctgctgaccctgctatgcacgctgcttctggtaatctattact

SEQ ID NO: 16 - RNA, 3178 nt, synthetic construct
  source 1..3178: mol_type = other RNA
tggagtcacattaattggagaagccgtaaaaacacagttcaattattataagaaagttgatggtgttgtccaacaattacctgaaacttactttactcagagtagaaatttacaagaatttaaacccaggagtcaaatggaaattgatttcttagaattagctatggatgaattcattgaacggtataaattagaaggctatgccttcgaacatatcgtttatggagattttagtcatagtcagttaggtgggttacatttacttatagggttagctaaaagatttaaagaatcaccattcgaactcgaagactttatacctatggatagtacggttaagaattattttattactgacgctcaaaccggttcatctaaatgcgtttgttcagttatagacttactgttagacgattttgtcgaaattattaagtctcaggatctatcagtcgtatctaaagtcgttaaggttacaatcgattatactgagatatcttttatgttatggtgtaaagacggtcacgttgagactttttatcctaaattgcaatctagtcaagcttggcaacccggtgtcgctatgcctaatctatataaaatgcaacgtatgttactcgaaaaatgcgatttacagaattacggtgattccgctacattgcctaaaggtattatgatgaatgtcgctaaatatacacaattgtgtcaatatcttaatacacttacacttgcagttccatataatatgagagtgatacattttggcgcaggatctgataagggagtcgcaccaggtactgccgtacttagacaatggttacctacaggtacactgttagtcgattccgatcttaacgattttgtttctgacgctgattctacacttataggcgattgtgctacagtgcataccgctaataaatgggatcttattatatccgatatgtacgatcctaaaactaaaaacgttactaaggaaaacgattctaaagagggtttttttacttatatttgtggttttatacagcaaaaattagcgttaggcggatccgttgcgattaagattaccgaacatagttggaatgctgatctatataagcttatgggtcatttcgcatggtggactgcattcgttacgaatgttaacgcttctagttccgaagcttttttaatcggatgtaattatttaggtaagcctagggaacagattgacggatacgttatgcatgctaattatattttttggcgtaatactaatcctattcaattgtctagttattcattattcgatatgtctaaatttccacttaaacttaggggtactgccgttatgtcacttaaggaaggtcaaattaacgatatgatactatcattgttatctaaaggtagattgattataagagaaaacaacagagttgttatttctagtgatgttcttgttaacaactaaacgaacaatgtttgtttttcttgttttattgccactagtctctagtcagtgtgttaatcttacaaccagaactcaattaccccctgcatacactaattctttcacacgtggtgtttattaccctgacaaagttttcagatcctcagttttacattcaactcaggacttgttcttacctttcttttccaatgttacttggttccatgctatacatgtctctgggaccaatggtactaagaggtttgataaccctgtcctaccatttaatgatggtgtttattttgcttccactgagaagtctaacataataagaggctggatttttggtactactttagattcgaagacccagtccctacttattgttaataacgctactaatgttgttattaaagtctgtgaatttcaattttgtaatgatccatttttgggtgtttattaccacaaaaacaacaaaagttggatggaaagtgagttcagagtttattctagtgcgaataattgcacttttgaatatgtctctcagccttttcttatggaccttgaaggaaaacagggtaatttcaaaaatcttagggaatttgtgtttaagaatattgatggttattttaaaatatattctaagcacacgcctattaatttagtgcgtgatctccctcagggtttttcggctttagaaccattggtagatttgccaataggtattaacatcactaggtttcaaactttacttgctttacatagaagttatttgactcctggtgattcttcttcaggttggacagctggtgctgcagcttattatgtgggttatcttcaacctaggacttttctattaaaatataatgaaaatggaaccattacagatgctgtagactgtgcacttgaccctctctcagaaacaaagtgtacgttgaaatccttcactgtagaaaaaggaatctatcaaacttctaactttagagtccaaccaacagaatctattgttagatttcctaatattacaaacttgtgcccttttggtgaagtttttaacgccaccagatttgcatctgtttatgcttggaacaggaagagaatcagcaactgtgttgctgattattctgtcctatataattccgcatcattttccacttttaagtgttatggagtgtctcctactaaattaaatgatctctgctttactaatgtctatgcagattcatttgtaattagaggtgatgaagtcagacaaatcgctccagggcaaactggaaagattgctgattataattataaattaccagatgattttacaggctgcgttatagcttggaattctaacaatcttgattctaaggttggtggtaattataattacctgtatagattgtttaggaagtctaatctcaaaccttttgagagagatatttcaactgaaatctatcaggccggtagcacaccttgtaatggtgttgaaggttttaattgttactttcctttacaatcatatggtttccaacccactaatggtgttggttaccaaccatacagagtagtagtactttcttttgaacttctacatgcaccagcaactgtttgtggacctaaaaagtctactaatttggttaaaaacaaatgtgtcaatttcaacttcaatggtttaacaggcacaggtgttcttactgagtctaacaaaaagtttctgcctttccaacaatttggcagagacattgctgacactactgatgc

SEQ ID NO: 17 - RNA, 2966 nt, synthetic construct
  source 1..2966: mol_type = other RNA
aatctatcaggccggtagcacaccttgtaatggtgttgaaggttttaattgttactttcctttacaatcatatggtttccaacccactaatggtgttggttaccaaccatacagagtagtagtactttcttttgaacttctacatgcaccagcaactgtttgtggacctaaaaagtctactaatttggttaaaaacaaatgtgtcaatttcaacttcaatggtttaacaggcacaggtgttcttactgagtctaacaaaaagtttctgcctttccaacaatttggcagagacattgctgacactactgatgctgtccgtgatccacagacacttgagattcttgacattacaccatgttcttttggtggtgtcagtgttataacaccaggaacaaatacttctaaccaggttgctgttctttatcaggatgttaactgcacagaagtccctgttgctattcatgcagatcaacttactcctacttggcgtgtttattctacaggttctaatgtttttcaaacacgtgcaggctgtttaataggggctgaacatgtcaacaactcatatgagtgtgacatacccattggtgcaggtatatgcgctagttatcagactcagactaattctcctcggcgggcacgtagtgtagctagtcaatccatcattgcctacactatgtcacttggtgcagaaaattcagttgcttactctaataactctattgccatacccacaaattttactattagtgttaccacagaaattctaccagtgtctatgaccaagacatcagtagattgtacaatgtacatttgtggtgattcaactgaatgcagcaatcttttgttgcaatatggcagtttttgtacacaattaaaccgtgctttaactggaatagctgttgaacaagacaaaaacacccaagaagtttttgcacaagtcaaacaaatttacaaaacaccaccaattaaagattttggtggttttaatttttcacaaatattaccagatccatcaaaaccaagcaagaggtcatttattgaagatctacttttcaacaaagtgacacttgcagatgctggcttcatcaaacaatatggtgattgccttggtgatattgctgctagagacctcatttgtgcacaaaagtttaacggccttactgttttgccacctttgctcacagatgaaatgattgctcaatacacttctgcactgttagcgggtacaatcacttctggttggacctttggtgcaggtgctgcattacaaataccatttgctatgcaaatggcttataggtttaatggtattggagttacacagaatgttctctatgagaaccaaaaattgattgccaaccaatttaattccgctataggtaagattcaagactcattgtctagtaccgctagtgcattaggtaagttgcaagacgtcgttaaccaaaacgctcaagcacttaatacacttgttaagcaattgtctagtaattttggcgctattagttcagtgcttaacgatattctatcacgtcttgataaagtcgaagccgaagtgcaaatcgatagattgattaccggtagattgcaatctcttcaaacttatgttacacaacaattgattagggctgccgaaattagggctagtgctaatctcgcagctactaaaatgtctgaatgcgtactcggtcaatctaaacgtgtcgatttttgcggtaagggatatcatcttatgtcttttccacaatccgcaccacatggagtggtttttttacacgttacatacgttccagctcaggaaaaaaattttactaccgcaccagctatttgtcatgacggtaaggcacattttcctagagagggagtattcgtttctaacggtacacattggttcgttacacaacgtaatttttacgagccacaaattattactactgataatacattcgttagcggtaattgcgacgtagtgataggtatagttaataatacagtttacgatccattgcaacctgaactcgattcttttaaagaggaactcgataagtattttaaaaaccatacatcacctgacgttgacttaggcgatatttccggtattaacgctagcgtagttaatattcaaaaagaaattgatagacttaacgaagtcgctaaaaaccttaacgaatcacttatcgatcttcaagagttaggtaagtatgagcaatatattaaatggccttggtatatttggttagggtttatagccggtcttatcgcaatcgttatggttacaattatgttatgttgtatgacatcatgttgttcatgtcttaagggatgttgttcatgcggatcatgttgtaaatttgacgaagacgactctgagccagtgctcaaaggagtcaaattacattacacataaacgaacttatggatttgtttatgagaatcttcacaattggaactgtaactttgaagcaaggtgaaatcaaggatgctactccttcagattttgttcgcgctactgcaacgataccgatacaagcctcactccctttcggatggcttattgttggcgttgcacttcttgctgtttttcagagcgcttccaaaatcataaccctcaaaaagagatggcaactagcactctccaagggtgttcactttgtttgcaacttgctgttgttgtttgtaacagtttactcacaccttttgctcgttgctgctggccttgaagccccttttctctatctttatgctttagtctacttcttgcagagtataaactttgtaagaataataatgaggctttggctttgctggaaatgccgttccaaaaacccattactttatgatgccaactattttctttgctggcatactaattgttacgactattgtataccttacaatagtgtaacttcttcaattgtcattacttcaggtgatggcacaacaagtcctatttctgaacatga

SEQ ID NO: 18 - RNA, 24 nt, synthetic construct
  source 1..24: mol_type = other RNA
attctcctcggcgggcacgtagtg

SEQ ID NO: 19 - RNA, 29875 nt, synthetic construct
  source 1..29875: mol_type = other RNA
atattaggtttataccttcccaggtaacaaaccaaccaactttcgatctcttgtagatctgttctctaaacgaactttaaaatctgtgtggctgtcactcggctgcatgcttagtgcactcacgcagtataattaataactaattactgtcgttgacaggacacgagtaactcgtctatcttctgcaggctgcttacggtttcgtccgtgttgcagccgatcatcagcacatctaggtttcgtccgggtgtgaccgaaaggtaagatggagagccttgtccctggtttcaacgagaaaacacacgtccaactcagtttgcctgttttacaggttcgcgacgtgctcgtacgtggctttggagactccgtggaggaggtcttatcagaggcacgtcaacatcttaaagatggcacttgtggcttagtagaagttgaaaaaggcgttttgcctcaacttgaacagccctatgtgttcatcaaacgttcggatgctcgaactgcacctcatggtcatgttatggttgagctggtagcagaactcgaaggcattcagtacggtcgtagtggtgagacacttggtgtccttgtccctcatgtgggcgaaataccagtggcttaccgcaaggttcttcttcgtaagaacggtaataaaggagctggtggccatagttacggcgccgatctaaagtcatttgacttaggcgacgagcttggcactgatccttatgaagattttcaagaaaactggaacactaaacatagcagtggtgttacccgtgaactcatgcgtgagcttaacggaggggcatacactcgctatgtcgataacaacttctgtggccctgatggctaccctcttgagtgcattaaagaccttctagcacgtgctggtaaagcttcatgcactttgtccgaacaactggactttattgacactaagaggggtgtatactgctgccgtgaacatgagcatgaaattgcttggtacacggaacgttctgaaaagagctatgaattgcagacaccttttgaaattaaattggcaaagaaatttgacaccttcaatggggaatgtccaaattttgtatttcccttaaattccataatcaagactattcaaccaagggttgaaaagaaaaagcttgatggctttatgggtagaattcgatctgtctatccagttgcgtcaccaaatgaatgcaaccaaatgtgcctttcaactctcatgaagtgtgatcattgtggtgaaacttcatggcagacgggcgattttgttaaagccacttgcgaattttgtggcactgagaatttgactaaagaaggtgccactacttgtggttacttaccccaaaatgctgttgttaaaatttattgtccagcatgtcacaattcagaagtaggacctgagcatagtcttgccgaataccataatgaatctggcttgaaaaccattcttcgtaagggtggtcgcactattgcctttggaggctgtgtgttctcttatgttggttgccataacaagtgtgcctattgggttccacgtgctagcgctaacataggttgtaaccatacaggtgttgttggagaaggttccgaaggtcttaatgacaaccttcttgaaatactccaaaaagagaaagtcaacatcaatattgttggtgactttaaacttaatgaagagatcgccattattttggcatctttttctgcttccacaagtgcttttgtggaaactgtgaaaggtttggattataaagcattcaaacaaattgttgaatcctgtggtaattttaaagttacaaaaggaaaagctaaaaaaggtgcctggaatattggtgaacagaaatcaatactgagtcctctttatgcatttgcatcagaggctgctcgtgttgtacgatcaattttctcccgcactcttgaaactgctcaaaattctgtgcgtgttttacagaaggccgctataacaatactagatggaatttcacagtattcactgagactcattgatgctatgatgttcacatctgatttggctactaacaatctagttgtaatggcctacattacaggtggtgttgttcagttgacttcgcagtggctaactaacatctttggcactgtttatgaaaaactcaaacccgtccttgattggcttgaagagaagtttaaggaaggtgtagagtttcttagagacggttgggaaattgttaaatttatctcaacctgtgcttgtgaaattgtcggtggacaaattgtcacctgtgcaaaggaaattaaggagagtgttcagacattctttaagcttgtaaataaatttttggctttgtgtgctgactctatcattattggtggagctaaacttaaagccttgaatttaggtgaaacatttgtcacgcactcaaagggattgtacagaaagtgtgttaaatccagagaagaaactggcctactcatgcctctaaaagccccaaaagaaattatcttcttagagggagaaacacttcccacagaagtgttaacagaggaagttgtcttgaaaactggtgatttacaaccattagaacaacctactagtgaagctgttgaagctccattggttggtacaccagtttgtattaacgggcttatgttgctcgaaatcaaagacacagaaaagtactgtgcccttgcacctaatatgatggtaacaaacaataccttcacactcaaaggcggtgcaccaacaaaggttacttttggtgatgacactgtgatagaagtgcaaggttacaagagtgtgaatatcacttttgaacttgatgaaaggattgataaagtacttaatgagaagtgctctgcctatacagttgaactcggtacagaagtaaatgagttcgcctgtgttgtggcagatgctgtcataaaaactttgcaaccagtatctgaattacttacaccactgggcattgatttagatgagtggagtatggctacatactacttatttgatgagtctggtgagtttaaattggcttcacatatgtattgttctttctaccctccagatgaggatgaagaagaaggtgattgtgaagaagaagagtttgagccatcaactcaatatgagtatggtactgaagatgattaccaaggtaaacctttggaatttggtgccacttctgctgctcttcaacctgaagaagagcaagaagaagattggttagatgatgatagtcaacaaactgttggtcaacaagacggcagtgaggacaatcagacaactactattcaaacaattgttgaggttcaacctcaattagagatggaacttacaccagttgttcagactattgaagtgaatagttttagtggttatttaaaacttactgacaatgtatacattaaaaatgcagacattgtggaagaagctaaaaaggtaaaaccaacagtggttgttaatgcagccaatgtttaccttaaacatggaggaggtgttgcaggagccttaaataaggctactaacaatgccatgcaagttgaatctgatgattacatagctactaatggaccacttaaagtgggtggtagttgtgttttaagcggacacaatcttgctaaacactgtcttcatgttgtcggcccaaatgttaacaaaggtgaagacattcaacttcttaagagtgcttatgaaaattttaatcagcacgaagttctacttgcaccattattatcagctggtatttttggtgctgaccctatacattctttaagagtttgtgtagatactgttcgcacaaatgtctacttagctgtctttgataaaaatctctatgacaaacttgtttcaagctttttggaaatgaagagtgaaaagcaagttgaacaaaagatcgctgagattcctaaagaggaagttaagccatttataactgaaagtaaaccttcagttgaacagagaaaacaagatgataagaaaatcaaagcttgtgttgaagaagttacaacaactctggaagaaactaagttcctcacagaaaacttgttactttatattgacattaatggcaatcttcatccagattctgccactcttgttagtgacattgacatcactttcttaaagaaagatgctccatatatagtgggtgatgttgttcaagagggtgttttaactgctgtggttatacctactaaaaaggctggtggcactactgaaatgctagcgaaagctttgagaaaagtgccaacagacaattatataaccacttacccgggtcagggtttaaatggttacactgtagaggaggcaaagacagtgcttaaaaagtgtaaaagtgccttttacattctaccatctattatctctaatgagaagcaagaaattcttggaactgtttcttggaatttgcgagaaatgcttgcacatgcagaagaaacacgcaaattaatgcctgtctgtgtggaaactaaagccatagtttcaactatacagcgtaaatataagggtattaaaatacaagagggtgtggttgattatggtgctagattttacttttacaccagtaaaacaactgtagcgtcacttatcaacacacttaacgatctaaatgaaactcttgttacaatgccacttggctatgtaacacatggcttaaatttggaagaagctgctcggtatatgagatctctcaaagtgccagctacagtttctgtttcttcacctgatgctgttacagcgtataatggttatcttacttcttcttctaaaacacctgaagaacattttattgaaaccatctcacttgctggttcctataaagattggtcctattctggacaatctacacaactaggtatagaatttcttaagagaggtgataaaagtgtatattacactagtaatcctaccacattccacctagatggtgaagttatcacctttgacaatcttaagacacttctttctttgagagaagtgaggactattaaggtgtttacaacagtagacaacattaacctccacacgcaagttgtggacatgtcaatgacatatggacaacagtttggtccaacttatttggatggagctgatgttactaaaataaaacctcataattcacatgaaggtaaaacattttatgttttacctaatgatgacactctacgtgttgaggcttttgagtactaccacacaactgatcctagttttctgggtaggtacatgtcagcattaaatcacactaaaaagtggaaatacccacaagttaatggtttaacttctattaaatgggcagataacaactgttatcttgccactgcattgttaacactccaacaaatagagttgaagtttaatccacctgctctacaagatgcttattacagagcaagggctggtgaagctgctaacttttgtgcacttatcttagcctactgtaataagacagtaggtgagttaggtgatgttagagaaacaatgagttacttgtttcaacatgccaatttagattcttgcaaaagagtcttgaacgtggtgtgtaaaacttgtggacaacagcagacaacccttaagggtgtagaagctgttatgtacatgggcacactttcttatgaacaatttaagaaaggtgttcagataccttgtacgtgtggtaaacaagctacaaaatatctagtacaacaggagtcaccttttgttatgatgtcagcaccacctgctcagtatgaacttaagcatggtacatttacttgtgctagtgagtacactggtaattaccagtgtggtcactataaacatataacttctaaagaaactttgtattgcatagacggtgctttacttacaaagtcctcagaatacaaaggtcctattacggatgttttctacaaagaaaacagttacacaacaaccataaaaccagttacttataaattggatggtgttgtttgtacagaaattgaccctaagttggacaattattataagaaagacaattcttatttcacagagcaaccaattgatcttgtaccaaaccaaccatatccaaacgcaagcttcgataattttaagtttgtatgtgataatatcaaatttgctgatgatttaaaccagttaactggttataagaaacctgcttcaagagagcttaaagttacatttttccctgacttaaatggtgatgtggtggctattgattataaacactacacaccctcttttaagaaaggagctaaattgttacataaacctattgtttggcatgttaacaatgcaactaataaagccacgtataaaccaaatacctggtgtatacgttgtctttggagcacaaaaccagttgaaacatcaaattcgtttgatgtactgaagtcagaggacgcgcagggaatggataatcttgcctgcgaagatctaaaaccagtctctgaagaagtagtggaaaatcctaccatacagaaagacgttcttgagtgtaatgtgaaaactaccgaagttgtaggagacattatacttaaaccagcaaataatagtttaaaaattacagaagaggttggccacacagatctaatggctgcttatgtagacaattctagtcttactattaagaaacctaatgaattatctagagtattaggtttgaaaacccttgctactcatggtttagctgctgttaatagtgtcccttgggatactatagctaattatgctaagccttttcttaacaaagttgttagtacaactactaacatagttacacggtgtttaaaccgtgtttgtactaattatatgccttatttctttactttattgctacaattgtgtacttttactagaagtacaaattctagaattaaagcatctatgccgactactatagcaaagaatactgttaagagtgtcggtaaattttgtctagaggcttcatttaattatttgaagtcacctaatttttctaaactgataaatattataatttggtttttactattaagtgtttgcctaggttctttaatctactcaaccgctgctttaggtgttttaatgtctaatttaggcatgccttcttactgtactggttacagagaaggctatttgaactctactaatgtcactattgcaacctactgtactggttctataccttgtagtgtttgtcttagtggtttagattctttagacacctatccttctttagaaactatacaaattaccatttcatcttttaaatgggatttaactgcttttggcttagttgcagagtggtttttggcatatattcttttcactaggtttttctatgtacttggattggctgcaatcatgcaattgtttttcagctattttgcagtacattttattagtaattcttggcttatgtggttaataattaatcttgtacaaatggccccgatttcagctatggttagaatgtacatcttctttgcatcattttattatgtatggaaaagttatgtgcatgttgtagacggttgtaattcatcaacttgtatgatgtgttacaaacgtaatagagcaacaagagtcgaatgtacaactattgttaatggtgttagaaggtccttttatgtctatgctaatggaggtaaaggcttttgcaaactacacaattggaattgtgttaattgtgatacattctgtgctggtagtacatttattagtgatgaagttgcgagagacttgtcactacagtttaaaagaccaataaatcctactgaccagtcttcttacatcgttgatagtgttacagtgaagaatggttccatccatctttactttgataaagctggtcaaaagacttatgaaagacattctctctctcattttgttaacttagacaacctgagagctaataacactaaaggttcattgcctattaatgttatagtttttgatggtaaatcaaaatgtgaagaatcatctgcaaaatcagcgtctgtttactacagtcagcttatgtgtcaacctatactgttactagatcaggcattagtgtctgatgttggtgatagtgcggaagttgcagttaaaatgtttgatgcttacgttaatacgttttcatcaacttttaacgtaccaatggaaaaactcaaaacactagttgcaactgcagaagctgaacttgcaaagaatgtgtccttagacaatgtcttatctacttttatttcagcagctcggcaagggtttgttgattcagatgtagaaactaaagatgttgttgaatgtcttaaattgtcacatcaatctgacatagaagttactggcgatagttgtaataactatatgctcacctataacaaagttgaaaacatgacaccccgtgaccttggtgcttgtattgactgtagtgcgcgtcatattaatgcgcaggtagcaaaaagtcacaacattgctttgatatggaacgttaaagatttcatgtcattgtctgaacaactacgaaaacaaatacgtagtgctgctaaaaagaataacttaccttttaagttgacatgtgcaactactagacaagttgttaatgttgtaacaacaaagatagcacttaagggtggtaaaattgttaataattggttgaagcagttaattaaagttacacttgtgttcctttttgttgctgctattttctatttaataacacctgttcatgtcatgtctaaacatactgacttttcaagtgaaatcataggatacaaggctattgatggtggtgtcactcgtgacatagcatctacagatacttgttttgctaacaaacatgctgattttgacacatggtttagccagcgtggtggtagttatactaatgacaaagcttgcccattgattgctgcagtcataacaagagaagtgggttttgtcgtgcctggtttgcctggcacgatattacgcacaactaatggtgactttttgcatttcttacctagagtttttagtgcagttggtaacatctgttacacaccatcaaaacttatagagtacactgactttgcaacatcagcttgtgttttggctgctgaatgtacaatttttaaagatgcttctggtaagccagtaccatattgttatgataccaatgtactagaaggttctgttgcttatgaaagtttacgccctgacacacgttatgtgctcatggatggctctattattcaatttcctaacacctaccttgaaggttctgttagagtggtaacaacttttgattctgagtactgtaggcacggcacttgtgaaagatcagaagctggtgtttgtgtatctactagtggtagatgggtacttaacaatgattattacagatctttaccaggagttttctgtggtgtagatgctgtaaatttacttactaatatgtttacaccactaattcaacctattggtgctttggacatatcagcatctatagtagctggtggtattgtagctatcgtagtaacatgccttgcctactattttatgaggtttagaagagcttttggtgaatacagtcatgtagttgcctttaatactttactattccttatgtcattcactgtactctgtttaacaccagtttactcattcttacctggtgtttattctgttatttacttgtacttgacattttatcttactaatgatgtttcttttttagcacatattcagtggatggttatgttcacacctttagtacctttctggataacaattgcttatatcatttgtatttccacaaagcatttctattggttctttagtaattacctaaagagacgtgtagtctttaatggtgtttcctttagtacttttgaagaagctgcgctgtgcacctttttgttaaataaagaaatgtatctaaagttgcgtagtgatgtgctattacctcttacgcaatataatagatacttagctctttataataagtacaagtattttagtggagcaatggatacaactagctacagagaagctgcttgttgtcatctcgcaaaggctctcaatgacttcagtaactcaggttctgatgttctttaccaaccaccacaaacctctatcacctcagctgttttgcagagtggttttagaaaaatggcattcccatctggtaaagttgagggttgtatggtacaagtaacttgtggtacaactacacttaacggtctttggcttgatgacgtagtttactgtccaagacatgtgatctgcacctctgaagacatgcttaaccctaattatgaagatttactcattcgtaagtctaatcataatttcttggtacaggctggtaatgttcaactcagggttattggacattctatgcaaaattgtgtacttaagcttaaggttgatacagccaatcctaagacacctaagtataagtttgttcgcattcaaccaggacagactttttcagtgttagcttgttacaatggttcaccatctggtgtttaccaatgtgctatgaggcccaatttcactattaagggttcattccttaatggttcatgtggtagtgttggttttaacatagattatgactgtgtctctttttgttacatgcaccatatggaattaccaactggagttcatgctggcacagacttagaaggtaacttttatggaccttttgttgacaggcaaacagcacaagcagctggtacggacacaactattacagttaatgttttagcttggttgtacgctgctgttataaatggagacaggtggtttctcaatcgatttaccacaactcttaatgactttaaccttgtggctatgaagtacaattatgaacctctaacacaagaccatgttgacatactaggacctctttctgctcaaactggaattgccgttttagatatgtgtgcttcattaaaagaattactgcaaaatggtatgaatggacgtaccatattgggtagtgctttattagaagatgaatttacaccttttgatgttgttagacaatgctcaggtgttactttccaaagtgcagtgaaaagaacaatcaagggtacacaccactggttgttactcacaattttgacttcacttttagttttagtccagagtactcaatggtctttgttcttttttttgtatgaaaatgcctttttaccttttgctatgggtattattgctatgtctgcttttgcaatgatgtttgtcaaacataagcatgcatttctctgtttgtttttgttaccttctcttgccactgtagcttattttaatatggtctatatgcctgctagttgggtgatgcgtattatgacatggttggatatggttgatactagtttgtctggttttaagctaaaagactgtgttatgtatgcatcagctgtagtgttactaatccttatgacagcaagaactgtgtatgatgatggtgctaggagagtgtggacacttatgaatgtcttgacactcgtttataaagtttattatggtaatgctttagatcaagccatttccatgtgggctcttataatctctgttacttctaactactcaggtgtagttacaactgtcatgtttttggccagaggtattgtttttatgtgtgttgagtattgccctattttcttcataactggtaatacacttcagtgtataatgctagtttattgtttcttaggctatttttgtacttgttactttggcctcttttgtttactcaaccgctactttagactgactcttggtgtttatgattacttagtttctacacaggagtttagatatatgaattcacagggactactcccacccaagaatagcatagatgccttcaaactcaacattaaattgttgggtgttggtggcaaaccttgtatcaaagtagccactgtacagtctaaaatgtcagatgtaaagtgcacatcagtagtcttactctcagttttgcaacaactcagagtagaatcatcatctaaattgtgggctcaatgtgtccagttacacaatgacattctcttagctaaagatactactgaagcctttgaaaaaatggtttcactactttctgttttgctttccatgcagggtgctgtagacataaacaagctttgtgaagaaatgctggacaacagggcaaccttacaagctatagcctcagagtttagttcccttccatcatatgcagcttttgctactgctcaagaagcttatgagcaggctgttgctaatggtgattctgaagttgttcttaaaaagttgaagaagtctttgaatgtggctaaatctgaatttgaccgtgatgcagccatgcaacgtaagttggaaaagatggctgatcaagctatgacccaaatgtataaacaggctagatctgaggacaagagggcaaaagttactagtgctatgcagacaatgcttttcactatgcttagaaagttggataatgatgcactcaacaacattatcaacaatgcaagagatggttgtgttcccttgaacataatacctcttacaacagcagccaaactaatggttgtcataccagactataacacatataaaaatacgtgtgatggtacaacatttacttatgcatcagcattgtgggaaatccaacaggttgtagatgcagatagtaaaattgttcaacttagtgaaattagtatggacaattcacctaatttagcatggcctcttattgtaacagctttaagggccaattctgctgtcaaattacagaataatgagcttagtcctgttgcactacgacagatgtcttgtgctgccggtactacacaaactgcttgcactgatgacaatgcgttagcttactacaacacaacaaagggaggtaggtttgtacttgcactgttatccgatttacaggatttgaaatgggctagattccctaagagtgatggaactggtactatctatacagaactggaaccaccttgtaggtttgttacagacacacctaaaggtcctaaagtgaagtatttatactttattaaaggattaaacaacctaaatagaggtatggtacttggtagtttagctgccacagtacgtctacaagctggtaatgcaacagaagtgcctgccaattcaactgtattatctttctgtgcttttgctgtagatgctgctaaagcttacaaagattatctagctagtgggggacaaccaatcactaattgtgttaagatgttgtgtacacacactggtactggtcaggcaataacagttacaccggaagccaatatggatcaagaatcctttggtggtgcatcgtgttgtctgtactgccgttgccacatagatcatccaaatcctaaaggattttgtgacttaaaaggtaagtatgtacaaatacctacaacttgtgctaatgaccctgtgggttttacacttaaaaacacagtctgtaccgtctgcggtatgtggaaaggttatggctgtagttgtgatcaactccgcgaacccatgcttcagtcagctgatgcacaatcgtttttaaacgggtttgcggtgtaagtgcagcccgtcttacaccgtgcggcacaggcactagtactgatgtcgtatacagggcttttgacatctacaatgataaagtagctggttttgctaaattcctaaaaactaattgttgtcgcttccaagaaaaggacgaagatgacaatttaattgattcttactttgtagttaagagacacactttctctaactaccaacatgaagaaacaatttataatttacttaaggattgtccagctgttgctaaacatgacttctttaagtttagaatagacggtgacatggtaccacatatatcacgtcaacgtcttactaaatacacaatggcagacctcgtctatgctttaaggcattttgatgaaggtaattgtgacacattaaaagaaatacttgtcacatacaattgttgtgatgatgattatttcaataaaaaggactggtatgattttgtagaaaacccagatatattacgcgtatacgccaacttaggtgaacgtgtacgccaagctttgttaaaaacagtacaattctgtgatgccatgcgaaatgctggtattgttggtgtactgacattagataatcaagatctcaatggtaactggtatgatttcggtgatttcatacaaaccacgccaggtagtggagttcctgttgtagattcttattattcattgttaatgcctatattaaccttgaccagggctttaactgcagagtcacatgttgacactgacttaacaaagccttacattaagtgggatttgttaaaatatgacttcacggaagagaggttaaaactctttgaccgttattttaaatattgggatcagacataccacccaaattgtgttaactgtttggatgacagatgcattctgcattgtgcaaactttaatgttttattctctacagtgttcccacctacaagttttggaccactagtgagaaaaatatttgttgatggtgttccatttgtagtttcaactggataccacttcagagagctaggtgttgtacataatcaggatgtaaacttacatagctctagacttagttttaaggaattacttgtgtatgctgctgaccctgctatgcacgctgcttctggtaatctattactagataaacgcactacgtgcttttcagtagctgcacttactaacaatgttgcttttcaaactgtcaaacccggtaattttaacaaagacttctatgactttgctgtgtctaagggtttctttaaggaaggaagttctgttgaattaaaacacttcttctttgctcaggatggtaatgctgctatcagcgattatgactactatcgttataatctaccaacaatgtgtgatatcagacaactactatttgtagttgaagttgttgataagtactttgattgttacgatggtggctgtattaatgctaaccaagtcatcgtcaacaacctagacaaatcagctggttttccatttaataaatggggtaaggctagactttattatgattcaatgagttatgaggatcaagatgcacttttcgcatatacaaaacgtaatgtcatccctactataactcaaatgaatcttaagtatgccattagtgcaaagaatagagctcgcaccgtagctggtgtctctatctgtagtactatgaccaatagacagtttcatcaaaaattattgaaatcaatagccgccactagaggagctactgtagtaattggaacaagcaaattctatggtggttggcacaacatgttaaaaactgtttatagtgatgtagaaaaccctcaccttatgggttgggattatcctaaatgtgatagagccatgcctaacatgcttagaattatggcctcacttgttcttgctcgcaaacatacaacgtgttgtagcttgtcacaccgtttctatagattagctaatgagtgtgctcaagtattgagtgaaatggtcatgtgtggcggttcactatatgttaaaccaggtggaacctcatcaggagatgccacaactgcttatgctaatagtgtttttaacatttgtcaagctgtcacggccaatgttaatgcacttttatctactgatggtaacaaaattgccgataagtatgtccgcaatttacaacacagactttatgagtgtctctatagaaatagagatgttgacacagactttgtgaatgagttttacgcatatttgcgtaaacatttctcaatgatgatactctctgacgatgctgttgtgtgtttcaatagcacttatgcatctcaaggtctagtggctagcataaagaactttaagtcagttctttattatcaaaacaatgtttttatgtctgaagcaaaatgttggactgagactgaccttactaaaggacctcatgaattttgctctcaacatacaatgctagttaaacagggtgatgattatgtgtaccttccttacccagatccatcaagaatcctaggggccggctgttttgtagatgatatcgtaaaaacagatggtacacttatgattgaacggttcgtgtctttagctatagatgcttacccacttactaaacatcctaatcaggagtatgctgatgtctttcatttgtacttacaatacataagaaagctacatgatgagttaacaggacacatgttagacatgtattctgttatgcttactaatgataacacttcaaggtattgggaacctgagttttatgaggctatgtacacaccgcatacagtcttacaggctgttggggcttgtgttctttgcaattcacagacttcattaagatgtggtgcttgcatacgtagaccattcttatgttgtaaatgctgttacgaccatgtcatatcaacatcacataaattagtcttgtctgttaatccgtatgtttgcaatgctccaggttgtgatgtcacagatgtgactcaactttacttaggaggtatgagctattattgtaaatcacataaaccacccattagttttccattgtgtgctaatggacaagtttttggtttatataaaaatacatgtgttggtagcgataatgttactgactttaatgcaattgcaacatgtgactggacaaatgctggtgattacattttagctaacacctgtactgaaagactcaagctttttgcagcagaaacgctcaaagctactgaggagacatttaaactgtcttatggtattgctactgtacgtgaagtgctgtctgacagagaattacatctttcatgggaagttggtaaacctagaccaccacttaaccgaaattatgtctttactggttatcgtgtaactaaaaacagtaaagtacaaataggagagtacacctttgaaaaaggtgactatggtgatgctgttgtttaccgaggtacaacaacttacaaattaaatgttggtgattattttgtgctgacatcacatacagtaatgccattaagtgcacctacactagtgccacaagagcactatgttagaattactggcttatacccaacactcaatatctcagatgagttttctagcaatgttgcaaattatcaaaaggttggtatgcaaaagtattctacactccagggaccacctggtactggtaagagtcattttgctattggcctagctctctactacccttctgctcgcatagtgtatacagcttgctctcatgccgctgttgatgcactatgtgagaaggcattaaaatatttgcctatagataaatgtagtagaattatacctgcacgtgctcgtgtagagtgttttgataaattcaaagtgaattcaacattagaacagtatgtcttttgtactgtaaatgcattgcctgagacgacagcagatatagttgtctttgatgaaatttcaatggccacaaattatgatttgagtgttgtcaatgccagattacgtgctaagcactatgtgtacattggcgaccctgctcaattacctgcaccacgcacattgctaactaagggcacactagaaccagaatatttcaattcagtgtgtagacttatgaaaactataggtccagacatgttcctcggaacttgtcggcgttgtcctgctgaaattgttgacactgtgagtgctttggtttatgataataagcttaaagcacataaagacaaatcagctcaatgctttaaaatgttttataagggtgttatcacgcatgatgtttcatctgcaattaacaggccacaaataggcgtggtaagagaattccttacacgtaaccctgcttggagaaaagctgtctttatttcaccttataattcacagaatgctgtagcctcaaagattttgggactaccaactcaaactgttgattcatcacagggctcagaatatgactatgtcatattcactcaaaccactgaaacagctcactcttgtaatgtaaacagatttaatgttgctattaccagagcaaaagtaggcatactttgcataatgtctgatagagacctttatgacaagttgcaatttacaagtcttgaaattccacgtaggaatgtggcaactttacaagctgaaaatgtaacaggactctttaaagattgtagtaaggtaatcactgggttacatcctacacaggcacctacacacctcagtgttgacactaaattcaaaactgaaggtttatgtgttgacatacctggcatacctaaggacatgacctatagaagactcatctctatgatgggttttaaaatgaattatcaagttaatggttaccctaacatgtttatcacccgcgaagaagctataagacatgtacgtgcatggattggcttcgatgtcgaggggtgtcatgctactagagaagctgttggtaccaatttacctttacagctaggtttttctacaggtgttaacctagttgctgtacctacaggttatgttgatacacctaataatacagatttttccagagttagtgctaaaccaccgcctggagatcaatttaaacacctcataccacttatgtacaaaggacttccttggaatgtagtgcgtataaagattgtacaaatgttaagtgacacacttaaaaatctctctgacagagtcgtatttgtcttatgggcacatggctttgagttgacatctatgaagtattttgtgaaaataggacctgagcgcacctgttgtctatgtgatagacgtgccacatgcttttccactgcttcagacacttatgcctgttggcatcattctattggatttgattacgtctataatccgtttatgattgatgttcaacaatggggttttacaggtaacctacaaagcaaccatgatctgtattgtcaagtccatggtaatgcacatgtagctagttgtgatgcaatcatgactaggtgtctagctgtccacgagtgctttgttaagcgtgttgactggactattgaatatcctataattggtgatgaactgaagattaatgcggcttgtagaaaggttcaacacatggttgttaaagctgcattattagcagacaaattcccagttcttcacgacattggtaaccctaaagctattaagtgtgtacctcaagctgatgtagaatggaagttctatgatgcacagccttgtagtgacaaagcttataaaatagaagaattattctattcttatgccacacattctgacaaattcacagatggtgtatgcctattttggaattgcaatgtcgatagatatcctgctaattccattgtttgtagatttgacactagagtgctatctaaccttaacttgcctggttgtgatggtggcagtttgtatgtaaataaacatgcattccacacaccagcttttgataaaagtgcttttgttaatttaaaacaattaccatttttctattactctgacagtccatgtgagtctcatggaaaacaagtagtgtcagatatagattatgtaccactaaagtctgctacgtgtataacacgttgcaatttaggtggtgctgtctgtagacatcatgctaatgagtacagattgtatctcgatgcttataacatgatgatctcagctggctttagcttgtgggtttacaaacaatttgatacttataacctctggaacacttttacaagacttcagagtttagaaaatgtggcttttaatgttgtaaataagggacactttgatggacaacagggtgaagtaccagtttctatcattaataacactgtttacacaaaagttgatggtgttgatgtagaattgtttgaaaataaaacaacattacctgttaatgtagcatttgagctttgggctaagcgcaacattaaaccagtaccagaggtgaaaatactcaataatttgggtgtggacattgctgctaatactgtgatctgggactacaaaagagatgctccagcacatatatctactattggtgtttgttctatgactgacatagccaagaaaccaactgaaacgatttgtgcaccactcactgtcttttttgatggtagagttgatggtcaagtagacttatttagaaatgcccgtaatggtgttcttattacagaaggtagtgttaaaggtttacaaccatctgtaggtcccaaacaagctagtcttaatggagtcacattaattggagaagccgtaaaaacacagttcaattattataagaaagttgatggtgttgtccaacaattacctgaaacttactttactcagagtagaaatttacaagaatttaaacccaggagtcaaatggaaattgatttcttagaattagctatggatgaattcattgaacggtataaattagaaggctatgccttcgaacatatcgtttatggagattttagtcatagtcagttaggtgggttacatttacttatagggttagctaaaagatttaaagaatcaccattcgaactcgaagactttatacctatggatagtacggttaagaattattttattactgacgctcaaaccggttcatctaaatgcgtttgttcagttatagacttactgttagacgattttgtcgaaattattaagtctcaggatctatcagtcgtatctaaagtcgttaaggttacaatcgattatactgagatatcttttatgttatggtgtaaagacggtcacgttgagactttttatcctaaattgcaatctagtcaagcttggcaacccggtgtcgctatgcctaatctatataaaatgcaacgtatgttactcgaaaaatgcgatttacagaattacggtgattccgctacattgcctaaaggtattatgatgaatgtcgctaaatatacacaattgtgtcaatatcttaatacacttacacttgcagttccatataatatgagagtgatacattttggcgcaggatctgataagggagtcgcaccaggtactgccgtacttagacaatggttacctacaggtacactgttagtcgattccgatcttaacgattttgtttctgacgctgattctacacttataggcgattgtgctacagtgcataccgctaataaatgggatcttattatatccgatatgtacgatcctaaaactaaaaacgttactaaggaaaacgattctaaagagggtttttttacttatatttgtggttttatacagcaaaaattagcgttaggcggatccgttgcgattaagattaccgaacatagttggaatgctgatctatataagcttatgggtcatttcgcatggtggactgcattcgttacgaatgttaacgcttctagttccgaagcttttttaatcggatgtaattatttaggtaagcctagggaacagattgacggatacgttatgcatgctaattatattttttggcgtaatactaatcctattcaattgtctagttattcattattcgatatgtctaaatttccacttaaacttaggggtactgccgttatgtcacttaaggaaggtcaaattaacgatatgatactatcattgttatctaaaggtagattgattataagagaaaacaacagagttgttatttctagtgatgttcttgttaacaactaaacgaacaatgtttgtttttcttgttttattgccactagtctctagtcagtgtgttaatcttacaaccagaactcaattaccccctgcatacactaattctttcacacgtggtgtttattaccctgacaaagttttcagatcctcagttttacattcaactcaggacttgttcttacctttcttttccaatgttacttggttccatgctatacatgtctctgggaccaatggtactaagaggtttgataaccctgtcctaccatttaatgatggtgtttattttgcttccactgagaagtctaacataataagaggctggatttttggtactactttagattcgaagacccagtccctacttattgttaataacgctactaatgttgttattaaagtctgtgaatttcaattttgtaatgatccatttttgggtgtttattaccacaaaaacaacaaaagttggatggaaagtgagttcagagtttattctagtgcgaataattgcacttttgaatatgtctctcagccttttcttatggaccttgaaggaaaacagggtaatttcaaaaatcttagggaatttgtgtttaagaatattgatggttattttaaaatatattctaagcacacgcctattaatttagtgcgtgatctccctcagggtttttcggctttagaaccattggtagatttgccaataggtattaacatcactaggtttcaaactttacttgctttacatagaagttatttgactcctggtgattcttcttcaggttggacagctggtgctgcagcttattatgtgggttatcttcaacctaggacttttctattaaaatataatgaaaatggaaccattacagatgctgtagactgtgcacttgaccctctctcagaaacaaagtgtacgttgaaatccttcactgtagaaaaaggaatctatcaaacttctaactttagagtccaaccaacagaatctattgttagatttcctaatattacaaacttgtgcccttttggtgaagtttttaacgccaccagatttgcatctgtttatgcttggaacaggaagagaatcagcaactgtgttgctgattattctgtcctatataattccgcatcattttccacttttaagtgttatggagtgtctcctactaaattaaatgatctctgctttactaatgtctatgcagattcatttgtaattagaggtgatgaagtcagacaaatcgctccagggcaaactggaaagattgctgattataattataaattaccagatgattttacaggctgcgttatagcttggaattctaacaatcttgattctaaggttggtggtaattataattacctgtatagattgtttaggaagtctaatctcaaaccttttgagagagatatttcaactgaaatctatcaggccggtagcacaccttgtaatggtgttgaaggttttaattgttactttcctttacaatcatatggtttccaacccactaatggtgttggttaccaaccatacagagtagtagtactttcttttgaacttctacatgcaccagcaactgtttgtggacctaaaaagtctactaatttggttaaaaacaaatgtgtcaatttcaacttcaatggtttaacaggcacaggtgttcttactgagtctaacaaaaagtttctgcctttccaacaatttggcagagacattgctgacactactgatgctgtccgtgatccacagacacttgagattcttgacattacaccatgttcttttggtggtgtcagtgttataacaccaggaacaaatacttctaaccaggttgctgttctttatcaggatgttaactgcacagaagtccctgttgctattcatgcagatcaacttactcctacttggcgtgtttattctacaggttctaatgtttttcaaacacgtgcaggctgtttaataggggctgaacatgtcaacaactcatatgagtgtgacatacccattggtgcaggtatatgcgctagttatcagactcagactatagctagtcaatccatcattgcctacactatgtcacttggtgcagaaaattcagttgcttactctaataactctattgccatacccacaaattttactattagtgttaccacagaaattctaccagtgtctatgaccaagacatcagtagattgtacaatgtacatttgtggtgattcaactgaatgcagcaatcttttgttgcaatatggcagtttttgtacacaattaaaccgtgctttaactggaatagctgttgaacaagacaaaaacacccaagaagtttttgcacaagtcaaacaaatttacaaaacaccaccaattaaagattttggtggttttaatttttcacaaatattaccagatccatcaaaaccaagcaagaggtcatttattgaagatctacttttcaacaaagtgacacttgcagatgctggcttcatcaaacaatatggtgattgccttggtgatattgctgctagagacctcatttgtgcacaaaagtttaacggccttactgttttgccacctttgctcacagatgaaatgattgctcaatacacttctgcactgttagcgggtacaatcacttctggttggacctttggtgcaggtgctgcattacaaataccatttgctatgcaaatggcttataggtttaatggtattggagttacacagaatgttctctatgagaaccaaaaattgattgccaaccaatttaatagtgctattggcaaaattcaagactcactttcttccacagcaagtgcacttggaaaacttcaagatgtggtcaaccaaaatgcacaagctttaaacacgcttgttaaacaacttagctccaattttggtgcaatttcaagtgttttaaatgatatcctttcacgtcttgacaaagttgaggctgaagtgcaaattgataggttgatcacaggcagacttcaaagtttgcagacatatgtgactcaacaattaattagagctgcagaaatcagagcttctgctaatcttgctgctactaaaatgtcagagtgtgtacttggacaatcaaaaagagttgatttttgtggaaagggctatcatcttatgtccttccctcagtcagcacctcatggtgtagtcttcttgcatgtgacttatgtccctgcacaagaaaagaacttcacaactgctcctgccatttgtcatgatggaaaagcacactttcctcgtgaaggtgtctttgtttcaaatggcacacactggtttgtaacacaaaggaatttttatgaaccacaaatcattactacagacaacacatttgtgtctggtaactgtgatgttgtaataggaattgtcaacaacacagtttatgatcctttgcaacctgaattagactcattcaaggaggagttagataaatattttaagaatcatacatcaccagatgttgatttaggtgacatctctggcattaatgcttcagttgtaaacattcaaaaagaaattgaccgcctcaatgaggttgccaagaatttaaatgaatctctcatcgatctccaagaacttggaaagtatgagcagtatataaaatggccatggtacatttggctaggttttatagctggcttgattgccatagtaatggtgacaattatgctttgctgtatgaccagttgctgtagttgtctcaagggctgttgttcttgtggatcctgctgcaaatttgatgaagacgactctgagccagtgctcaaaggagtcaaattacattacacataaacgaacttatggatttgtttatgagaatcttcacaattggaactgtaactttgaagcaaggtgaaatcaaggatgctactccttcagattttgttcgcgctactgcaacgataccgatacaagcctcactccctttcggatggcttattgttggcgttgcacttcttgctgtttttcagagcgcttccaaaatcataaccctcaaaaagagatggcaactagcactctccaagggtgttcactttgtttgcaacttgctgttgttgtttgtaacagtttactcacaccttttgctcgttgctgctggccttgaagccccttttctctatctttatgctttagtctacttcttgcagagtataaactttgtaagaataataatgaggctttggctttgctggaaatgccgttccaaaaacccattactttatgatgccaactattttctttgctggcatactaattgttacgactattgtataccttacaatagtgtaacttcttcaattgtcattacttcaggtgatggcacaacaagtcctatttctgaacatgactaccagattggtggttatactgaaaaatgggaatctggagtaaaagactgtgttgtattacacagttacttcacttcagactattaccagctgtactcaactcaattgagtacagacactggtgttgaacatgttaccttcttcatctacaataaaattgttgatgagcctgaagaacatgtccaaattcacacaatcgacggttcatccggagttgttaatccagtaatggaaccaatttatgatgaaccgacgacgactactagcgtgcctttgtaagcacaagctgatgagtacgaacttatgtactcattcgtttcggaagagacaggtacgttaatagttaatagcgtacttctttttcttgctttcgtggtattcttgctagttacactagccatccttactgcgcttcgattgtgtgcgtactgctgcaatattgttaacgtgagtcttgtaaaaccttctttttacgtttactctcgtgttaaaaatctgaattcttctagagttcctgatcttctggtctaaacgaactaaatattatattagtttttctgtttggaactttaattttagccatggcagattccaacggtactattaccgttgaagagcttaaaaagctccttgaacaatggaacctagtaataggtttcctattccttacatggatttgtcttctacaatttgcctatgccaacaggaataggtttttgtatataattaagttaattttcctctggctgttatggccagtaactttagcttgttttgtgcttgctgctgtttacagaataaattggatcaccggtggaattgctatcgcaatggcttgtcttgtaggcttgatgtggctcagctacttcattgcttctttcagactgtttgcgcgtacgcgttccatgtggtcattcaatccagaaactaacattcttctcaacgtgccactccatggcactattctgaccagaccgcttctagaaagtgaactcgtaatcggagctgtgatccttcgtggacatcttcgtattgctggacaccatctaggacgctgtgacatcaaggacctgcctaaagaaatcactgttgctacatcacgaacgctttcttattacaaattgggagcttcgcagcgtgtagcaggtgactcaggttttgctgcatacagtcgctacaggattggcaactataaattaaacacagaccattccagtagcagtgacaatattgctttgcttgtacagtaagtgacaacagatgtttcatctcgttgactttcaggttactatagcagagatattactaattattatgaggacttttaaagtttccatttggaatcttgattacatcataaacctcataattaaaaatttatctaagtcactaactgagaataaatattctcaattagatgaagagcaaccaatggagattgattaaacgaacatgaaaattattcttttcttggcactgataacactcgctacttgtgagctttatcactaccaagagtgtgttagaggtacaacagtacttttaaaagaaccttgctcttctggaacatacgagggcaattcaccatttcatcctctagctgataacaaatttgcactgacttgctttagcactcaatttgcttttgcttgtcctgacggcgtaaaacacgtctatcagttacgtgccagatcagtttcacctaaactgttcatcagacaagaggaagttcaagaactttactctccaatttttcttattgttgcggcaatagtgtttataacactttgcttcacactcaaaagaaagacagaatgattgaactttcattaattgacttctatttgtgctttttagcctttctgctattccttgttttaattatgcttattatcttttggttctcacttgaactgcaagatcataatgaaacttgtcacgcctaaacgaacatgaaatttcttgttttcttaggaatcatcacaactgtagctgcatttcaccaagaatgtagtttacagtcatgtactcaacatcaaccatatgtagttgatgacccgtgtcctattcacttctattctaaatggtatattagagtaggagctagaaaatcagcacctttaattgaattgtgcgtggatgaggctggttctaaatcacccattcagtacatcgatatcggtaattatacagtttcctgtttaccttttacaattaattgccaggaacctaaattgggtagtcttgtagtgcgttgttcgttctatgaagactttttagagtatcatgacgttcgtgttgttttagatttcatctaaacgaacaaactaaaatgtctgataatggaccccaaaatcagcgaaatgcaccccgcattacgtttggtggaccctcagattcaactggcagtaaccagaatggagaacgcagtggggcgcgatcaaaacaacgtcggccccaaggtttacccaataatactgcgtcttggttcaccgctctcactcaacatggcaaggaagaccttaaattccctcgaggacaaggcgttccaattaacaccaatagcagtccagatgaccaaattggctactaccgaagagctaccagacgaattcgtggtggtgacggtaaaatgaaagatctcagtccaagatggtatttctactacctaggaactgggccagaagctggacttccctatggtgctaacaaagacggcatcatatgggttgcaactgagggagccttgaatacaccaaaagatcacattggcacccgcaatcctgctaacaatgctgcaatcgtgctacaacttcctcaaggaacaacattgccaaaaggcttctacgcagaagggagcagaggcggcagtcaagcctcttctcgttcctcatcacgtagtcgcaacagttcaagaaattcaactccaggcagcagtaggggaacttctcctgctagaatggctggcaatggcggtgatgctgctcttgctttgctgctgcttgacagattgaaccagcttgagagcaaaatgtctggtaaaggccaacaacaacaaggccaaactgtcactaagaaatctgctgctgaggcttctaagaagcctcggcaaaaacgtactgccactaaagcatacaatgtaacacaagctttcggcagacgtggtccagaacaaacccaaggaaattttggggaccaggaactaatcagacaaggaactgattacaaacattggccgcaaattgcacaatttgcccccagcgcttcagcgttcttcggaatgtcgcgcattggcatggaagtcacaccttcgggaacgtggttgacctacacaggtgccatcaaattggatgacaaagatccaaatttcaaagatcaagtcattttgctgaataagcatattgacgcatacaaaacattcccaccaacagagcctaaaaaggacaaaaagaagaaggctgatgaaactcaagccttaccgcagagacagaagaaacagcaaactgtgactcttcttcctgctgcagatttggatgatttctccaaacaattgcaacaatccatgagcagtgctgactcaactcaggcctaaactcatgcagaccacacaaggcagatgggctatataaacgttttcgcttttccgtttacgatatatagtctactcttgtgcagaatgaattctcgtaactacatagcacaagtagatgtagttaactttaatctcacatagcaatctttaatcagtgtgtaacattagggaggacttgaaagagccaccacattttcaccgaggccacgcggagtacgatcgagtgtacagtgaacaatgctagggagagctgcctatatggaagagccctaatgtgtaaaattaattttagtagtgctatccccatgtgattttaatagcttcttaggagaatgacaaaaaaaaaaaaaaaaaaaaaaaaaaaaa

SEQ ID NO: 20 - RNA, 29875 nt, synthetic construct
  source 1..29875: mol_type = other RNA
atattaggtttataccttcccaggtaacaaaccaaccaactttcgatctcttgtagatctgttctctaaacgaactttaaaatctgtgtggctgtcactcggctgcatgcttagtgcactcacgcagtataattaataactaattactgtcgttgacaggacacgagtaactcgtctatcttctgcaggctgcttacggtttcgtccgtgttgcagccgatcatcagcacatctaggtttcgtccgggtgtgaccgaaaggtaagatggagagccttgtccctggtttcaacgagaaaacacacgtccaactcagtttgcctgttttacaggttcgcgacgtgctcgtacgtggctttggagactccgtggaggaggtcttatcagaggcacgtcaacatcttaaagatggcacttgtggcttagtagaagttgaaaaaggcgttttgcctcaacttgaacagccctatgtgttcatcaaacgttcggatgctcgaactgcacctcatggtcatgttatggttgagctggtagcagaactcgaaggcattcagtacggtcgtagtggtgagacacttggtgtccttgtccctcatgtgggcgaaataccagtggcttaccgcaaggttcttcttcgtaagaacggtaataaaggagctggtggccatagttacggcgccgatctaaagtcatttgacttaggcgacgagcttggcactgatccttatgaagattttcaagaaaactggaacactaaacatagcagtggtgttacccgtgaactcatgcgtgagcttaacggaggggcatacactcgctatgtcgataacaacttctgtggccctgatggctaccctcttgagtgcattaaagaccttctagcacgtgctggtaaagcttcatgcactttgtccgaacaactggactttattgacactaagaggggtgtatactgctgccgtgaacatgagcatgaaattgcttggtacacggaacgttctgaaaagagctatgaattgcagacaccttttgaaattaaattggcaaagaaatttgacaccttcaatggggaatgtccaaattttgtatttcccttaaattccataatcaagactattcaaccaagggttgaaaagaaaaagcttgatggctttatgggtagaattcgatctgtctatccagttgcgtcaccaaatgaatgcaaccaaatgtgcctttcaactctcatgaagtgtgatcattgtggtgaaacttcatggcagacgggcgattttgttaaagccacttgcgaattttgtggcactgagaatttgactaaagaaggtgccactacttgtggttacttaccccaaaatgctgttgttaaaatttattgtccagcatgtcacaattcagaagtaggacctgagcatagtcttgccgaataccataatgaatctggcttgaaaaccattcttcgtaagggtggtcgcactattgcctttggaggctgtgtgttctcttatgttggttgccataacaagtgtgcctattgggttccacgtgctagcgctaacataggttgtaaccatacaggtgttgttggagaaggttccgaaggtcttaatgacaaccttcttgaaatactccaaaaagagaaagtcaacatcaatattgttggtgactttaaacttaatgaagagatcgccattattttggcatctttttctgcttccacaagtgcttttgtggaaactgtgaaaggtttggattataaagcattcaaacaaattgttgaatcctgtggtaattttaaagttacaaaaggaaaagctaaaaaaggtgcctggaatattggtgaacagaaatcaatactgagtcctctttatgcatttgcatcagaggctgctcgtgttgtacgatcaattttctcccgcactcttgaaactgctcaaaattctgtgcgtgttttacagaaggccgctataacaatactagatggaatttcacagtattcactgagactcattgatgctatgatgttcacatctgatttggctactaacaatctagttgtaatggcctacattacaggtggtgttgttcagttgacttcgcagtggctaactaacatctttggcactgtttatgaaaaactcaaacccgtccttgattggcttgaagagaagtttaaggaaggtgtagagtttcttagagacggttgggaaattgttaaatttatctcaacctgtgcttgtgaaattgtcggtggacaaattgtcacctgtgcaaaggaaattaaggagagtgttcagacattctttaagcttgtaaataaatttttggctttgtgtgctgactctatcattattggtggagctaaacttaaagccttgaatttaggtgaaacatttgtcacgcactcaaagggattgtacagaaagtgtgttaaatccagagaagaaactggcctactcatgcctctaaaagccccaaaagaaattatcttcttagagggagaaacacttcccacagaagtgttaacagaggaagttgtcttgaaaactggtgatttacaaccattagaacaacctactagtgaagctgttgaagctccattggttggtacaccagtttgtattaacgggcttatgttgctcgaaatcaaagacacagaaaagtactgtgcccttgcacctaatatgatggtaacaaacaataccttcacactcaaaggcggtgcaccaacaaaggttacttttggtgatgacactgtgatagaagtgcaaggttacaagagtgtgaatatcacttttgaacttgatgaaaggattgataaagtacttaatgagaagtgctctgcctatacagttgaactcggtacagaagtaaatgagttcgcctgtgttgtggcagatgctgtcataaaaactttgcaaccagtatctgaattacttacaccactgggcattgatttagatgagtggagtatggctacatactacttatttgatgagtctggtgagtttaaattggcttcacatatgtattgttctttctaccctccagatgaggatgaagaagaaggtgattgtgaagaagaagagtttgagccatcaactcaatatgagtatggtactgaagatgattaccaaggtaaacctttggaatttggtgccacttctgctgctcttcaacctgaagaagagcaagaagaagattggttagatgatgatagtcaacaaactgttggtcaacaagacggcagtgaggacaatcagacaactactattcaaacaattgttgaggttcaacctcaattagagatggaacttacaccagttgttcagactattgaagtgaatagttttagtggttatttaaaacttactgacaatgtatacattaaaaatgcagacattgtggaagaagctaaaaaggtaaaaccaacagtggttgttaatgcagccaatgtttaccttaaacatggaggaggtgttgcaggagccttaaataaggctactaacaatgccatgcaagttgaatctgatgattacatagctactaatggaccacttaaagtgggtggtagttgtgttttaagcggacacaatcttgctaaacactgtcttcatgttgtcggcccaaatgttaacaaaggtgaagacattcaacttcttaagagtgcttatgaaaattttaatcagcacgaagttctacttgcaccattattatcagctggtatttttggtgctgaccctatacattctttaagagtttgtgtagatactgttcgcacaaatgtctacttagctgtctttgataaaaatctctatgacaaacttgtttcaagctttttggaaatgaagagtgaaaagcaagttgaacaaaagatcgctgagattcctaaagaggaagttaagccatttataactgaaagtaaaccttcagttgaacagagaaaacaagatgataagaaaatcaaagcttgtgttgaagaagttacaacaactctggaagaaactaagttcctcacagaaaacttgttactttatattgacattaatggcaatcttcatccagattctgccactcttgttagtgacattgacatcactttcttaaagaaagatgctccatatatagtgggtgatgttgttcaagagggtgttttaactgctgtggttatacctactaaaaaggctggtggcactactgaaatgctagcgaaagctttgagaaaagtgccaacagacaattatataaccacttacccgggtcagggtttaaatggttacactgtagaggaggcaaagacagtgcttaaaaagtgtaaaagtgccttttacattctaccatctattatctctaatgagaagcaagaaattcttggaactgtttcttggaatttgcgagaaatgcttgcacatgcagaagaaacacgcaaattaatgcctgtctgtgtggaaactaaagccatagtttcaactatacagcgtaaatataagggtattaaaatacaagagggtgtggttgattatggtgctagattttacttttacaccagtaaaacaactgtagcgtcacttatcaacacacttaacgatctaaatgaaactcttgttacaatgccacttggctatgtaacacatggcttaaatttggaagaagctgctcggtatatgagatctctcaaagtgccagctacagtttctgtttcttcacctgatgctgttacagcgtataatggttatcttacttcttcttctaaaacacctgaagaacattttattgaaaccatctcacttgctggttcctataaagattggtcctattctggacaatctacacaactaggtatagaatttcttaagagaggtgataaaagtgtatattacactagtaatcctaccacattccacctagatggtgaagttatcacctttgacaatcttaagacacttctttctttgagagaagtgaggactattaaggtgtttacaacagtagacaacattaacctccacacgcaagttgtggacatgtcaatgacatatggacaacagtttggtccaacttatttggatggagctgatgttactaaaataaaacctcataattcacatgaaggtaaaacattttatgttttacctaatgatgacactctacgtgttgaggcttttgagtactaccacacaactgatcctagttttctgggtaggtacatgtcagcattaaatcacactaaaaagtggaaatacccacaagttaatggtttaacttctattaaatgggcagataacaactgttatcttgccactgcattgttaacactccaacaaatagagttgaagtttaatccacctgctctacaagatgcttattacagagcaagggctggtgaagctgctaacttttgtgcacttatcttagcctactgtaataagacagtaggtgagttaggtgatgttagagaaacaatgagttacttgtttcaacatgccaatttagattcttgcaaaagagtcttgaacgtggtgtgtaaaacttgtggacaacagcagacaacccttaagggtgtagaagctgttatgtacatgggcacactttcttatgaacaatttaagaaaggtgttcagataccttgtacgtgtggtaaacaagctacaaaatatctagtacaacaggagtcaccttttgttatgatgtcagcaccacctgctcagtatgaacttaagcatggtacatttacttgtgctagtgagtacactggtaattaccagtgtggtcactataaacatataacttctaaagaaactttgtattgcatagacggtgctttacttacaaagtcctcagaatacaaaggtcctattacggatgttttctacaaagaaaacagttacacaacaaccataaaaccagttacttataaattggatggtgttgtttgtacagaaattgaccctaagttggacaattattataagaaagacaattcttatttcacagagcaaccaattgatcttgtaccaaaccaaccatatccaaacgcaagcttcgataattttaagtttgtatgtgataatatcaaatttgctgatgatttaaaccagttaactggttataagaaacctgcttcaagagagcttaaagttacatttttccctgacttaaatggtgatgtggtggctattgattataaacactacacaccctcttttaagaaaggagctaaattgttacataaacctattgtttggcatgttaacaatgcaactaataaagccacgtataaaccaaatacctggtgtatacgttgtctttggagcacaaaaccagttgaaacatcaaattcgtttgatgtactgaagtcagaggacgcgcagggaatggataatcttgcctgcgaagatctaaaaccagtctctgaagaagtagtggaaaatcctaccatacagaaagacgttcttgagtgtaatgtgaaaactaccgaagttgtaggagacattatacttaaaccagcaaataatagtttaaaaattacagaagaggttggccacacagatctaatggctgcttatgtagacaattctagtcttactattaagaaacctaatgaattatctagagtattaggtttgaaaacccttgctactcatggtttagctgctgttaatagtgtcccttgggatactatagctaattatgctaagccttttcttaacaaagttgttagtacaactactaacatagttacacggtgtttaaaccgtgtttgtactaattatatgccttatttctttactttattgctacaattgtgtacttttactagaagtacaaattctagaattaaagcatctatgccgactactatagcaaagaatactgttaagagtgtcggtaaattttgtctagaggcttcatttaattatttgaagtcacctaatttttctaaactgataaatattataatttggtttttactattaagtgtttgcctaggttctttaatctactcaaccgctgctttaggtgttttaatgtctaatttaggcatgccttcttactgtactggttacagagaaggctatttgaactctactaatgtcactattgcaacctactgtactggttctataccttgtagtgtttgtcttagtggtttagattctttagacacctatccttctttagaaactatacaaattaccatttcatcttttaaatgggatttaactgcttttggcttagttgcagagtggtttttggcatatattcttttcactaggtttttctatgtacttggattggctgcaatcatgcaattgtttttcagctattttgcagtacattttattagtaattcttggcttatgtggttaataattaatcttgtacaaatggccccgatttcagctatggttagaatgtacatcttctttgcatcattttattatgtatggaaaagttatgtgcatgttgtagacggttgtaattcatcaacttgtatgatgtgttacaaacgtaatagagcaacaagagtcgaatgtacaactattgttaatggtgttagaaggtccttttatgtctatgctaatggaggtaaaggcttttgcaaactacacaattggaattgtgttaattgtgatacattctgtgctggtagtacatttattagtgatgaagttgcgagagacttgtcactacagtttaaaagaccaataaatcctactgaccagtcttcttacatcgttgatagtgttacagtgaagaatggttccatccatctttactttgataaagctggtcaaaagacttatgaaagacattctctctctcattttgttaacttagacaacctgagagctaataacactaaaggttcattgcctattaatgttatagtttttgatggtaaatcaaaatgtgaagaatcatctgcaaaatcagcgtctgtttactacagtcagcttatgtgtcaacctatactgttactagatcaggcattagtgtctgatgttggtgatagtgcggaagttgcagttaaaatgtttgatgcttacgttaatacgttttcatcaacttttaacgtaccaatggaaaaactcaaaacactagttgcaactgcagaagctgaacttgcaaagaatgtgtccttagacaatgtcttatctacttttatttcagcagctcggcaagggtttgttgattcagatgtagaaactaaagatgttgttgaatgtcttaaattgtcacatcaatctgacatagaagttactggcgatagttgtaataactatatgctcacctataacaaagttgaaaacatgacaccccgtgaccttggtgcttgtattgactgtagtgcgcgtcatattaatgcgcaggtagcaaaaagtcacaacattgctttgatatggaacgttaaagatttcatgtcattgtctgaacaactacgaaaacaaatacgtagtgctgctaaaaagaataacttaccttttaagttgacatgtgcaactactagacaagttgttaatgttgtaacaacaaagatagcacttaagggtggtaaaattgttaataattggttgaagcagttaattaaagttacacttgtgttcctttttgttgctgctattttctatttaataacacctgttcatgtcatgtctaaacatactgacttttcaagtgaaatcataggatacaaggctattgatggtggtgtcactcgtgacatagcatctacagatacttgttttgctaacaaacatgctgattttgacacatggtttagccagcgtggtggtagttatactaatgacaaagcttgcccattgattgctgcagtcataacaagagaagtgggttttgtcgtgcctggtttgcctggcacgatattacgcacaactaatggtgactttttgcatttcttacctagagtttttagtgcagttggtaacatctgttacacaccatcaaaacttatagagtacactgactttgcaacatcagcttgtgttttggctgctgaatgtacaatttttaaagatgcttctggtaagccagtaccatattgttatgataccaatgtactagaaggttctgttgcttatgaaagtttacgccctgacacacgttatgtgctcatggatggctctattattcaatttcctaacacctaccttgaaggttctgttagagtggtaacaacttttgattctgagtactgtaggcacggcacttgtgaaagatcagaagctggtgtttgtgtatctactagtggtagatgggtacttaacaatgattattacagatctttaccaggagttttctgtggtgtagatgctgtaaatttacttactaatatgtttacaccactaattcaacctattggtgctttggacatatcagcatctatagtagctggtggtattgtagctatcgtagtaacatgccttgcctactattttatgaggtttagaagagcttttggtgaatacagtcatgtagttgcctttaatactttactattccttatgtcattcactgtactctgtttaacaccagtttactcattcttacctggtgtttattctgttatttacttgtacttgacattttatcttactaatgatgtttcttttttagcacatattcagtggatggttatgttcacacctttagtacctttctggataacaattgcttatatcatttgtatttccacaaagcatttctattggttctttagtaattacctaaagagacgtgtagtctttaatggtgtttcctttagtacttttgaagaagctgcgctgtgcacctttttgttaaataaagaaatgtatctaaagttgcgtagtgatgtgctattacctcttacgcaatataatagatacttagctctttataataagtacaagtattttagtggagcaatggatacaactagctacagagaagctgcttgttgtcatctcgcaaaggctctcaatgacttcagtaactcaggttctgatgttctttaccaaccaccacaaacctctatcacctcagctgttttgcagagtggttttagaaaaatggcattcccatctggtaaagttgagggttgtatggtacaagtaacttgtggtacaactacacttaacggtctttggcttgatgacgtagtttactgtccaagacatgtgatctgcacctctgaagacatgcttaaccctaattatgaagatttactcattcgtaagtctaatcataatttcttggtacaggctggtaatgttcaactcagggttattggacattctatgcaaaattgtgtacttaagcttaaggttgatacagccaatcctaagacacctaagtataagtttgttcgcattcaaccaggacagactttttcagtgttagcttgttacaatggttcaccatctggtgtttaccaatgtgctatgaggcccaatttcactattaagggttcattccttaatggttcatgtggtagtgttggttttaacatagattatgactgtgtctctttttgttacatgcaccatatggaattaccaactggagttcatgctggcacagacttagaaggtaacttttatggaccttttgttgacaggcaaacagcacaagcagctggtacggacacaactattacagttaatgttttagcttggttgtacgctgctgttataaatggagacaggtggtttctcaatcgatttaccacaactcttaatgactttaaccttgtggctatgaagtacaattatgaacctctaacacaagaccatgttgacatactaggacctctttctgctcaaactggaattgccgttttagatatgtgtgcttcattaaaagaattactgcaaaatggtatgaatggacgtaccatattgggtagtgctttattagaagatgaatttacaccttttgatgttgttagacaatgctcaggtgttactttccaaagtgcagtgaaaagaacaatcaagggtacacaccactggttgttactcacaattttgacttcacttttagttttagtccagagtactcaatggtctttgttcttttttttgtatgaaaatgcctttttaccttttgctatgggtattattgctatgtctgcttttgcaatgatgtttgtcaaacataagcatgcatttctctgtttgtttttgttaccttctcttgccactgtagcttattttaatatggtctatatgcctgctagttgggtgatgcgtattatgacatggttggatatggttgatactagtttgtctggttttaagctaaaagactgtgttatgtatgcatcagctgtagtgttactaatccttatgacagcaagaactgtgtatgatgatggtgctaggagagtgtggacacttatgaatgtcttgacactcgtttataaagtttattatggtaatgctttagatcaagccatttccatgtgggctcttataatctctgttacttctaactactcaggtgtagttacaactgtcatgtttttggccagaggtattgtttttatgtgtgttgagtattgccctattttcttcataactggtaatacacttcagtgtataatgctagtttattgtttcttaggctatttttgtacttgttactttggcctcttttgtttactcaaccgctactttagactgactcttggtgtttatgattacttagtttctacacaggagtttagatatatgaattcacagggactactcccacccaagaatagcatagatgccttcaaactcaacattaaattgttgggtgttggtggcaaaccttgtatcaaagtagccactgtacagtctaaaatgtcagatgtaaagtgcacatcagtagtcttactctcagttttgcaacaactcagagtagaatcatcatctaaattgtgggctcaatgtgtccagttacacaatgacattctcttagctaaagatactactgaagcctttgaaaaaatggtttcactactttctgttttgctttccatgcagggtgctgtagacataaacaagctttgtgaagaaatgctggacaacagggcaaccttacaagctatagcctcagagtttagttcccttccatcatatgcagcttttgctactgctcaagaagcttatgagcaggctgttgctaatggtgattctgaagttgttcttaaaaagttgaagaagtctttgaatgtggctaaatctgaatttgaccgtgatgcagccatgcaacgtaagttggaaaagatggctgatcaagctatgacccaaatgtataaacaggctagatctgaggacaagagggcaaaagttactagtgctatgcagacaatgcttttcactatgcttagaaagttggataatgatgcactcaacaacattatcaacaatgcaagagatggttgtgttcccttgaacataatacctcttacaacagcagccaaactaatggttgtcataccagactataacacatataaaaatacgtgtgatggtacaacatttacttatgcatcagcattgtgggaaatccaacaggttgtagatgcagatagtaaaattgttcaacttagtgaaattagtatggacaattcacctaatttagcatggcctcttattgtaacagctttaagggccaattctgctgtcaaattacagaataatgagcttagtcctgttgcactacgacagatgtcttgtgctgccggtactacacaaactgcttgcactgatgacaatgcgttagcttactacaacacaacaaagggaggtaggtttgtacttgcactgttatccgatttacaggatttgaaatgggctagattccctaagagtgatggaactggtactatctatacagaactggaaccaccttgtaggtttgttacagacacacctaaaggtcctaaagtgaagtatttatactttattaaaggattaaacaacctaaatagaggtatggtacttggtagtttagctgccacagtacgtctacaagctggtaatgcaacagaagtgcctgccaattcaactgtattatctttctgtgcttttgctgtagatgctgctaaagcttacaaagattatctagctagtgggggacaaccaatcactaattgtgttaagatgttgtgtacacacactggtactggtcaggcaataacagttacaccggaagccaatatggatcaagaatcctttggtggtgcatcgtgttgtctgtactgccgttgccacatagatcatccaaatcctaaaggattttgtgacttaaaaggtaagtatgtacaaatacctacaacttgtgctaatgaccctgtgggttttacacttaaaaacacagtctgtaccgtctgcggtatgtggaaaggttatggctgtagttgtgatcaactccgcgaacccatgcttcagtcagctgatgcacaatcgtttttaaacgggtttgcggtgtaagtgcagcccgtcttacaccgtgcggcacaggcactagtactgatgtcgtatacagggcttttgacatctacaatgataaagtagctggttttgctaaattcctaaaaactaattgttgtcgcttccaagaaaaggacgaagatgacaatttaattgattcttactttgtagttaagagacacactttctctaactaccaacatgaagaaacaatttataatttacttaaggattgtccagctgttgctaaacatgacttctttaagtttagaatagacggtgacatggtaccacatatatcacgtcaacgtcttactaaatacacaatggcagacctcgtctatgctttaaggcattttgatgaaggtaattgtgacacattaaaagaaatacttgtcacatacaattgttgtgatgatgattatttcaataaaaaggactggtatgattttgtagaaaacccagatatattacgcgtatacgccaacttaggtgaacgtgtacgccaagctttgttaaaaacagtacaattctgtgatgccatgcgaaatgctggtattgttggtgtactgacattagataatcaagatctcaatggtaactggtatgatttcggtgatttcatacaaaccacgccaggtagtggagttcctgttgtagattcttattattcattgttaatgcctatattaaccttgaccagggctttaactgcagagtcacatgttgacactgacttaacaaagccttacattaagtgggatttgttaaaatatgacttcacggaagagaggttaaaactctttgaccgttattttaaatattgggatcagacataccacccaaattgtgttaactgtttggatgacagatgcattctgcattgtgcaaactttaatgttttattctctacagtgttcccacctacaagttttggaccactagtgagaaaaatatttgttgatggtgttccatttgtagtttcaactggataccacttcagagagctaggtgttgtacataatcaggatgtaaacttacatagctctagacttagttttaaggaattacttgtgtatgctgctgaccctgctatgcacgctgcttctggtaatctattactagataaacgcactacgtgcttttcagtagctgcacttactaacaatgttgcttttcaaactgtcaaacccggtaattttaacaaagacttctatgactttgctgtgtctaagggtttctttaaggaaggaagttctgttgaattaaaacacttcttctttgctcaggatggtaatgctgctatcagcgattatgactactatcgttataatctaccaacaatgtgtgatatcagacaactactatttgtagttgaagttgttgataagtactttgattgttacgatggtggctgtattaatgctaaccaagtcatcgtcaacaacctagacaaatcagctggttttccatttaataaatggggtaaggctagactttattatgattcaatgagttatgaggatcaagatgcacttttcgcatatacaaaacgtaatgtcatccctactataactcaaatgaatcttaagtatgccattagtgcaaagaatagagctcgcaccgtagctggtgtctctatctgtagtactatgaccaatagacagtttcatcaaaaattattgaaatcaatagccgccactagaggagctactgtagtaattggaacaagcaaattctatggtggttggcacaacatgttaaaaactgtttatagtgatgtagaaaaccctcaccttatgggttgggattatcctaaatgtgatagagccatgcctaacatgcttagaattatggcctcacttgttcttgctcgcaaacatacaacgtgttgtagcttgtcacaccgtttctatagattagctaatgagtgtgctcaagtattgagtgaaatggtcatgtgtggcggttcactatatgttaaaccaggtggaacctcatcaggagatgccacaactgcttatgctaatagtgtttttaacatttgtcaagctgtcacggccaatgttaatgcacttttatctactgatggtaacaaaattgccgataagtatgtccgcaatttacaacacagactttatgagtgtctctatagaaatagagatgttgacacagactttgtgaatgagttttacgcatatttgcgtaaacatttctcaatgatgatactctctgacgatgctgttgtgtgtttcaatagcacttatgcatctcaaggtctagtggctagcataaagaactttaagtcagttctttattatcaaaacaatgtttttatgtctgaagcaaaatgttggactgagactgaccttactaaaggacctcatgaattttgctctcaacatacaatgctagttaaacagggtgatgattatgtgtaccttccttacccagatccatcaagaatcctaggggccggctgttttgtagatgatatcgtaaaaacagatggtacacttatgattgaacggttcgtgtctttagctatagatgcttacccacttactaaacatcctaatcaggagtatgctgatgtctttcatttgtacttacaatacataagaaagctacatgatgagttaacaggacacatgttagacatgtattctgttatgcttactaatgataacacttcaaggtattgggaacctgagttttatgaggctatgtacacaccgcatacagtcttacaggctgttggggcttgtgttctttgcaattcacagacttcattaagatgtggtgcttgcatacgtagaccattcttatgttgtaaatgctgttacgaccatgtcatatcaacatcacataaattagtcttgtctgttaatccgtatgtttgcaatgctccaggttgtgatgtcacagatgtgactcaactttacttaggaggtatgagctattattgtaaatcacataaaccacccattagttttccattgtgtgctaatggacaagtttttggtttatataaaaatacatgtgttggtagcgataatgttactgactttaatgcaattgcaacatgtgactggacaaatgctggtgattacattttagctaacacctgtactgaaagactcaagctttttgcagcagaaacgctcaaagctactgaggagacatttaaactgtcttatggtattgctactgtacgtgaagtgctgtctgacagagaattacatctttcatgggaagttggtaaacctagaccaccacttaaccgaaattatgtctttactggttatcgtgtaactaaaaacagtaaagtacaaataggagagtacacctttgaaaaaggtgactatggtgatgctgttgtttaccgaggtacaacaacttacaaattaaatgttggtgattattttgtgctgacatcacatacagtaatgccattaagtgcacctacactagtgccacaagagcactatgttagaattactggcttatacccaacactcaatatctcagatgagttttctagcaatgttgcaaattatcaaaaggttggtatgcaaaagtattctacactccagggaccacctggtactggtaagagtcattttgctattggcctagctctctactacccttctgctcgcatagtgtatacagcttgctctcatgccgctgttgatgcactatgtgagaaggcattaaaatatttgcctatagataaatgtagtagaattatacctgcacgtgctcgtgtagagtgttttgataaattcaaagtgaattcaacattagaacagtatgtcttttgtactgtaaatgcattgcctgagacgacagcagatatagttgtctttgatgaaatttcaatggccacaaattatgatttgagtgttgtcaatgccagattacgtgctaagcactatgtgtacattggcgaccctgctcaattacctgcaccacgcacattgctaactaagggcacactagaaccagaatatttcaattcagtgtgtagacttatgaaaactataggtccagacatgttcctcggaacttgtcggcgttgtcctgctgaaattgttgacactgtgagtgctttggtttatgataataagcttaaagcacataaagacaaatcagctcaatgctttaaaatgttttataagggtgttatcacgcatgatgtttcatctgcaattaacaggccacaaataggcgtggtaagagaattccttacacgtaaccctgcttggagaaaagctgtctttatttcaccttataattcacagaatgctgtagcctcaaagattttgggactaccaactcaaactgttgattcatcacagggctcagaatatgactatgtcatattcactcaaaccactgaaacagctcactcttgtaatgtaaacagatttaatgttgctattaccagagcaaaagtaggcatactttgcataatgtctgatagagacctttatgacaagttgcaatttacaagtcttgaaattccacgtaggaatgtggcaactttacaagctgaaaatgtaacaggactctttaaagattgtagtaaggtaatcactgggttacatcctacacaggcacctacacacctcagtgttgacactaaattcaaaactgaaggtttatgtgttgacatacctggcatacctaaggacatgacctatagaagactcatctctatgatgggttttaaaatgaattatcaagttaatggttaccctaacatgtttatcacccgcgaagaagctataagacatgtacgtgcatggattggcttcgatgtcgaggggtgtcatgctactagagaagctgttggtaccaatttacctttacagctaggtttttctacaggtgttaacctagttgctgtacctacaggttatgttgatacacctaataatacagatttttccagagttagtgctaaaccaccgcctggagatcaatttaaacacctcataccacttatgtacaaaggacttccttggaatgtagtgcgtataaagattgtacaaatgttaagtgacacacttaaaaatctctctgacagagtcgtatttgtcttatgggcacatggctttgagttgacatctatgaagtattttgtgaaaataggacctgagcgcacctgttgtctatgtgatagacgtgccacatgcttttccactgcttcagacacttatgcctgttggcatcattctattggatttgattacgtctataatccgtttatgattgatgttcaacaatggggttttacaggtaacctacaaagcaaccatgatctgtattgtcaagtccatggtaatgcacatgtagctagttgtgatgcaatcatgactaggtgtctagctgtccacgagtgctttgttaagcgtgttgactggactattgaatatcctataattggtgatgaactgaagattaatgcggcttgtagaaaggttcaacacatggttgttaaagctgcattattagcagacaaattcccagttcttcacgacattggtaaccctaaagctattaagtgtgtacctcaagctgatgtagaatggaagttctatgatgcacagccttgtagtgacaaagcttataaaatagaagaattattctattcttatgccacacattctgacaaattcacagatggtgtatgcctattttggaattgcaatgtcgatagatatcctgctaattccattgtttgtagatttgacactagagtgctatctaaccttaacttgcctggttgtgatggtggcagtttgtatgtaaataaacatgcattccacacaccagcttttgataaaagtgcttttgttaatttaaaacaattaccatttttctattactctgacagtccatgtgagtctcatggaaaacaagtagtgtcagatatagattatgtaccactaaagtctgctacgtgtataacacgttgcaatttaggtggtgctgtctgtagacatcatgctaatgagtacagattgtatctcgatgcttataacatgatgatctcagctggctttagcttgtgggtttacaaacaatttgatacttataacctctggaacacttttacaagacttcagagtttagaaaatgtggcttttaatgttgtaaataagggacactttgatggacaacagggtgaagtaccagtttctatcattaataacactgtttacacaaaagttgatggtgttgatgtagaattgtttgaaaataaaacaacattacctgttaatgtagcatttgagctttgggctaagcgcaacattaaaccagtaccagaggtgaaaatactcaataatttgggtgtggacattgctgctaatactgtgatctgggactacaaaagagatgctccagcacatatatctactattggtgtttgttctatgactgacatagccaagaaaccaactgaaacgatttgtgcaccactcactgtcttttttgatggtagagttgatggtcaagtagacttatttagaaatgcccgtaatggtgttcttattacagaaggtagtgttaaaggtttacaaccatctgtaggtcccaaacaagctagtcttaatggagtcacattaattggagaagccgtaaaaacacagttcaattattataagaaagttgatggtgttgtccaacaattacctgaaacttactttactcagagtagaaatttacaagaatttaaacccaggagtcaaatggaaattgatttcttagaattagctatggatgaattcattgaacggtataaattagaaggctatgccttcgaacatatcgtttatggagattttagtcatagtcagttaggtggtttacatctactgattggactagctaaacgttttaaggaatcaccttttgaattagaagattttattcctatggacagtacagttaaaaactatttcataacagatgcgcaaacaggttcatctaagtgtgtgtgttctgttattgatttattacttgatgattttgttgaaataataaaatcccaagatttatctgtagtttctaaggttgtcaaagtgactattgactatacagaaatttcatttatgctttggtgtaaagatggccatgtagaaacattttacccaaaattacaatctagtcaagcgtggcaaccgggtgttgctatgcctaatctttacaaaatgcaaagaatgctattagaaaagtgtgaccttcaaaattatggtgatagtgcaacattacctaaaggcataatgatgaatgtcgcaaaatatactcaactgtgtcaatatttaaacacattaacattagctgtaccctataatatgagagttatacattttggtgctggttctgataaaggagttgcaccaggtacagctgttttaagacagtggttgcctacgggtacgctgcttgtcgattcagatcttaatgactttgtctctgatgcagattcaactttgattggtgattgtgcaactgtacatacagctaataaatgggatctcattattagtgatatgtacgaccctaagactaaaaatgttacaaaagaaaatgactctaaagagggttttttcacttacatttgtgggtttatacaacaaaagctagctcttggaggttccgtggctataaagataacagaacattcttggaatgctgatctttataagctcatgggacacttcgcatggtggacagcctttgttactaatgtgaatgcgtcatcatctgaagcatttttaattggatgtaattatcttggcaaaccacgcgaacaaatagatggttatgtcatgcatgcaaattacatattttggaggaatacaaatccaattcagttgtcttcctattctttatttgacatgagtaaatttccccttaaattaaggggtactgctgttatgtctttaaaagaaggtcaaatcaatgatatgattttatctcttcttagtaaaggtagacttataattagagaaaacaacagagttgttatttctagtgatgttcttgttaacaactaaacgaacaatgtttgtttttcttgttttattgccactagtctctagtcagtgtgttaatcttacaaccagaactcaattaccccctgcatacactaattctttcacacgtggtgtttattaccctgacaaagttttcagatcctcagttttacattcaactcaggacttgttcttacctttcttttccaatgttacttggttccatgctatacatgtctctgggaccaatggtactaagaggtttgataaccctgtcctaccatttaatgatggtgtttattttgcttccactgagaagtctaacataataagaggctggatttttggtactactttagattcgaagacccagtccctacttattgttaataacgctactaatgttgttattaaagtctgtgaatttcaattttgtaatgatccatttttgggtgtttattaccacaaaaacaacaaaagttggatggaaagtgagttcagagtttattctagtgcgaataattgcacttttgaatatgtctctcagccttttcttatggaccttgaaggaaaacagggtaatttcaaaaatcttagggaatttgtgtttaagaatattgatggttattttaaaatatattctaagcacacgcctattaatttagtgcgtgatctccctcagggtttttcggctttagaaccattggtagatttgccaataggtattaacatcactaggtttcaaactttacttgctttacatagaagttatttgactcctggtgattcttcttcaggttggacagctggtgctgcagcttattatgtgggttatcttcaacctaggacttttctattaaaatataatgaaaatggaaccattacagatgctgtagactgtgcacttgaccctctctcagaaacaaagtgtacgttgaaatccttcactgtagaaaaaggaatctatcaaacttctaactttagagtccaaccaacagaatctattgttagatttcctaatattacaaacttgtgcccttttggtgaagtttttaacgccaccagatttgcatctgtttatgcttggaacaggaagagaatcagcaactgtgttgctgattattctgtcctatataattccgcatcattttccacttttaagtgttatggagtgtctcctactaaattaaatgatctctgctttactaatgtctatgcagattcatttgtaattagaggtgatgaagtcagacaaatcgctccagggcaaactggaaagattgctgattataattataaattaccagatgattttacaggctgcgttatagcttggaattctaacaatcttgattctaaggttggtggtaattataattacctgtatagattgtttaggaagtctaatctcaaaccttttgagagagatatttcaactgaaatctatcaggccggtagcacaccttgtaatggtgttgaaggttttaattgttactttcctttacaatcatatggtttccaacccactaatggtgttggttaccaaccatacagagtagtagtactttcttttgaacttctacatgcaccagcaactgtttgtggacctaaaaagtctactaatttggttaaaaacaaatgtgtcaatttcaacttcaatggtttaacaggcacaggtgttcttactgagtctaacaaaaagtttctgcctttccaacaatttggcagagacattgctgacactactgatgctgtccgtgatccacagacacttgagattcttgacattacaccatgttcttttggtggtgtcagtgttataacaccaggaacaaatacttctaaccaggttgctgttctttatcaggatgttaactgcacagaagtccctgttgctattcatgcagatcaacttactcctacttggcgtgtttattctacaggttctaatgtttttcaaacacgtgcaggctgtttaataggggctgaacatgtcaacaactcatatgagtgtgacatacccattggtgcaggtatatgcgctagttatcagactcagactatagctagtcaatccatcattgcctacactatgtcacttggtgcagaaaattcagttgcttactctaataactctattgccatacccacaaattttactattagtgttaccacagaaattctaccagtgtctatgaccaagacatcagtagattgtacaatgtacatttgtggtgattcaactgaatgcagcaatcttttgttgcaatatggcagtttttgtacacaattaaaccgtgctttaactggaatagctgttgaacaagacaaaaacacccaagaagtttttgcacaagtcaaacaaatttacaaaacaccaccaattaaagattttggtggttttaatttttcacaaatattaccagatccatcaaaaccaagcaagaggtcatttattgaagatctacttttcaacaaagtgacacttgcagatgctggcttcatcaaacaatatggtgattgccttggtgatattgctgctagagacctcatttgtgcacaaaagtttaacggccttactgttttgccacctttgctcacagatgaaatgattgctcaatacacttctgcactgttagcgggtacaatcacttctggttggacctttggtgcaggtgctgcattacaaataccatttgctatgcaaatggcttataggtttaatggtattggagttacacagaatgttctctatgagaaccaaaaattgattgccaaccaatttaattccgctataggtaagattcaagactcattgtctagtaccgctagtgcattaggtaagttgcaagacgtcgttaaccaaaacgctcaagcacttaatacacttgttaagcaattgtctagtaattttggcgctattagttcagtgcttaacgatattctatcacgtcttgataaagtcgaagccgaagtgcaaatcgatagattgattaccggtagattgcaatctcttcaaacttatgttacacaacaattgattagggctgccgaaattagggctagtgctaatctcgcagctactaaaatgtctgaatgcgtactcggtcaatctaaacgtgtcgatttttgcggtaagggatatcatcttatgtcttttccacaatccgcaccacatggagtggtttttttacacgttacatacgttccagctcaggaaaaaaattttactaccgcaccagctatttgtcatgacggtaaggcacattttcctagagagggagtattcgtttctaacggtacacattggttcgttacacaacgtaatttttacgagccacaaattattactactgataatacattcgttagcggtaattgcgacgtagtgataggtatagttaataatacagtttacgatccattgcaacctgaactcgattcttttaaagaggaactcgataagtattttaaaaaccatacatcacctgacgttgacttaggcgatatttccggtattaacgctagcgtagttaatattcaaaaagaaattgatagacttaacgaagtcgctaaaaaccttaacgaatcacttatcgatcttcaagagttaggtaagtatgagcaatatattaaatggccttggtatatttggttagggtttatagccggtcttatcgcaatcgttatggttacaattatgttatgttgtatgacatcatgttgttcatgtcttaagggatgttgttcatgcggatcatgttgtaaatttgacgaagacgactctgagccagtgctcaaaggagtcaaattacattacacataaacgaacttatggatttgtttatgagaatcttcacaattggaactgtaactttgaagcaaggtgaaatcaaggatgctactccttcagattttgttcgcgctactgcaacgataccgatacaagcctcactccctttcggatggcttattgttggcgttgcacttcttgctgtttttcagagcgcttccaaaatcataaccctcaaaaagagatggcaactagcactctccaagggtgttcactttgtttgcaacttgctgttgttgtttgtaacagtttactcacaccttttgctcgttgctgctggccttgaagccccttttctctatctttatgctttagtctacttcttgcagagtataaactttgtaagaataataatgaggctttggctttgctggaaatgccgttccaaaaacccattactttatgatgccaactattttctttgctggcatactaattgttacgactattgtataccttacaatagtgtaacttcttcaattgtcattacttcaggtgatggcacaacaagtcctatttctgaacatgactaccagattggtggttatactgaaaaatgggaatctggagtaaaagactgtgttgtattacacagttacttcacttcagactattaccagctgtactcaactcaattgagtacagacactggtgttgaacatgttaccttcttcatctacaataaaattgttgatgagcctgaagaacatgtccaaattcacacaatcgacggttcatccggagttgttaatccagtaatggaaccaatttatgatgaaccgacgacgactactagcgtgcctttgtaagcacaagctgatgagtacgaacttatgtactcattcgtttcggaagagacaggtacgttaatagttaatagcgtacttctttttcttgctttcgtggtattcttgctagttacactagccatccttactgcgcttcgattgtgtgcgtactgctgcaatattgttaacgtgagtcttgtaaaaccttctttttacgtttactctcgtgttaaaaatctgaattcttctagagttcctgatcttctggtctaaacgaactaaatattatattagtttttctgtttggaactttaattttagccatggcagattccaacggtactattaccgttgaagagcttaaaaagctccttgaacaatggaacctagtaataggtttcctattccttacatggatttgtcttctacaatttgcctatgccaacaggaataggtttttgtatataattaagttaattttcctctggctgttatggccagtaactttagcttgttttgtgcttgctgctgtttacagaataaattggatcaccggtggaattgctatcgcaatggcttgtcttgtaggcttgatgtggctcagctacttcattgcttctttcagactgtttgcgcgtacgcgttccatgtggtcattcaatccagaaactaacattcttctcaacgtgccactccatggcactattctgaccagaccgcttctagaaagtgaactcgtaatcggagctgtgatccttcgtggacatcttcgtattgctggacaccatctaggacgctgtgacatcaaggacctgcctaaagaaatcactgttgctacatcacgaacgctttcttattacaaattgggagcttcgcagcgtgtagcaggtgactcaggttttgctgcatacagtcgctacaggattggcaactataaattaaacacagaccattccagtagcagtgacaatattgctttgcttgtacagtaagtgacaacagatgtttcatctcgttgactttcaggttactatagcagagatattactaattattatgaggacttttaaagtttccatttggaatcttgattacatcataaacctcataattaaaaatttatctaagtcactaactgagaataaatattctcaattagatgaagagcaaccaatggagattgattaaacgaacatgaaaattattcttttcttggcactgataacactcgctacttgtgagctttatcactaccaagagtgtgttagaggtacaacagtacttttaaaagaaccttgctcttctggaacatacgagggcaattcaccatttcatcctctagctgataacaaatttgcactgacttgctttagcactcaatttgcttttgcttgtcctgacggcgtaaaacacgtctatcagttacgtgccagatcagtttcacctaaactgttcatcagacaagaggaagttcaagaactttactctccaatttttcttattgttgcggcaatagtgtttataacactttgcttcacactcaaaagaaagacagaatgattgaactttcattaattgacttctatttgtgctttttagcctttctgctattccttgttttaattatgcttattatcttttggttctcacttgaactgcaagatcataatgaaacttgtcacgcctaaacgaacatgaaatttcttgttttcttaggaatcatcacaactgtagctgcatttcaccaagaatgtagtttacagtcatgtactcaacatcaaccatatgtagttgatgacccgtgtcctattcacttctattctaaatggtatattagagtaggagctagaaaatcagcacctttaattgaattgtgcgtggatgaggctggttctaaatcacccattcagtacatcgatatcggtaattatacagtttcctgtttaccttttacaattaattgccaggaacctaaattgggtagtcttgtagtgcgttgttcgttctatgaagactttttagagtatcatgacgttcgtgttgttttagatttcatctaaacgaacaaactaaaatgtctgataatggaccccaaaatcagcgaaatgcaccccgcattacgtttggtggaccctcagattcaactggcagtaaccagaatggagaacgcagtggggcgcgatcaaaacaacgtcggccccaaggtttacccaataatactgcgtcttggttcaccgctctcactcaacatggcaaggaagaccttaaattccctcgaggacaaggcgttccaattaacaccaatagcagtccagatgaccaaattggctactaccgaagagctaccagacgaattcgtggtggtgacggtaaaatgaaagatctcagtccaagatggtatttctactacctaggaactgggccagaagctggacttccctatggtgctaacaaagacggcatcatatgggttgcaactgagggagccttgaatacaccaaaagatcacattggcacccgcaatcctgctaacaatgctgcaatcgtgctacaacttcctcaaggaacaacattgccaaaaggcttctacgcagaagggagcagaggcggcagtcaagcctcttctcgttcctcatcacgtagtcgcaacagttcaagaaattcaactccaggcagcagtaggggaacttctcctgctagaatggctggcaatggcggtgatgctgctcttgctttgctgctgcttgacagattgaaccagcttgagagcaaaatgtctggtaaaggccaacaacaacaaggccaaactgtcactaagaaatctgctgctgaggcttctaagaagcctcggcaaaaacgtactgccactaaagcatacaatgtaacacaagctttcggcagacgtggtccagaacaaacccaaggaaattttggggaccaggaactaatcagacaaggaactgattacaaacattggccgcaaattgcacaatttgcccccagcgcttcagcgttcttcggaatgtcgcgcattggcatggaagtcacaccttcgggaacgtggttgacctacacaggtgccatcaaattggatgacaaagatccaaatttcaaagatcaagtcattttgctgaataagcatattgacgcatacaaaacattcccaccaacagagcctaaaaaggacaaaaagaagaaggctgatgaaactcaagccttaccgcagagacagaagaaacagcaaactgtgactcttcttcctgctgcagatttggatgatttctccaaacaattgcaacaatccatgagcagtgctgactcaactcaggcctaaactcatgcagaccacacaaggcagatgggctatataaacgttttcgcttttccgtttacgatatatagtctactcttgtgcagaatgaattctcgtaactacatagcacaagtagatgtagttaactttaatctcacatagcaatctttaatcagtgtgtaacattagggaggacttgaaagagccaccacattttcaccgaggccacgcggagtacgatcgagtgtacagtgaacaatgctagggagagctgcctatatggaagagccctaatgtgtaaaattaattttagtagtgctatccccatgtgattttaatagcttcttaggagaatgacaaaaaaaaaaaaaaaaaaaaaaaaaaaaa

SEQ ID NO: 21 - protein, 4 aa, synthetic construct
PRRA

SEQ ID NO: 22 - protein, 5 aa, synthetic construct
PRRAR

SEQ ID NO: 23 - protein, 6 aa, synthetic construct
PRRARS

SEQ ID NO: 24 - protein, 7 aa, synthetic construct
PRRARSV

SEQ ID NO: 25 - protein, 5 aa, synthetic construct
SPRRA

SEQ ID NO: 26 - protein, 6 aa, synthetic construct
SPRRAR

SEQ ID NO: 27 - protein, 7 aa, synthetic construct
SPRRARS

SEQ ID NO: 28 - protein, 8 aa, synthetic construct
SPRRARSV

SEQ ID NO: 29 - protein, 6 aa, synthetic construct
NSPRRA

SEQ ID NO: 30 - protein, 7 aa, synthetic construct
NSPRRAR

SEQ ID NO: 31 - protein, 8 aa, synthetic construct
NSPRRARS

SEQ ID NO: 32 - protein, 9 aa, synthetic construct
NSPRRARSV

SEQ ID NO: 33 - protein, 4 aa, synthetic construct
RRRA

SEQ ID NO: 34 - protein, 5 aa, synthetic construct
RRRAR

SEQ ID NO: 35 - protein, 6 aa, synthetic construct
RRRARS

SEQ ID NO: 36 - protein, 7 aa, synthetic construct
RRRARSV

SEQ ID NO: 37 - protein, 5 aa, synthetic construct
SRRRA

SEQ ID NO: 38 - protein, 6 aa, synthetic construct
SRRRAR

SEQ ID NO: 39 - protein, 7 aa, synthetic construct
SRRRARS

SEQ ID NO: 40 - protein, 8 aa, synthetic construct
SRRRARSV

SEQ ID NO: 41 - protein, 6 aa, synthetic construct
NSRRRA

SEQ ID NO: 42 - protein, 7 aa, synthetic construct
NSRRRAR

SEQ ID NO: 43 - protein, 8 aa, synthetic construct
NSRRRARS

SEQ ID NO: 44 - protein, 9 aa, synthetic construct
NSRRRARSV

SEQ ID NO: 45 - protein, 4 aa, synthetic construct
HRRA

SEQ ID NO: 46 - protein, 5 aa, synthetic construct
HRRAR

SEQ ID NO: 47 - protein, 6 aa, synthetic construct
HRRARS

SEQ ID NO: 48 - protein, 7 aa, synthetic construct
HRRARSV

SEQ ID NO: 49 - protein, 5 aa, synthetic construct
SHRRA

SEQ ID NO: 50 - protein, 6 aa, synthetic construct
SHRRAR

SEQ ID NO: 51 - protein, 7 aa, synthetic construct
SHRRARS

SEQ ID NO: 52 - protein, 8 aa, synthetic construct
SHRRARSV

SEQ ID NO: 53 - protein, 6 aa, synthetic construct
NSHRRA

SEQ ID NO: 54 - protein, 7 aa, synthetic construct
NSHRRAR

SEQ ID NO: 55 - protein, 8 aa, synthetic construct
NSHRRARS

SEQ ID NO: 56 - protein, 9 aa, synthetic construct
NSHRRARSV